European Patent Application EP 4 389 897 A1, published June 26, 2024. Title: POLYNUCLEOTIDE INCLUDING SITE-SPECIFIC NUCLEASE EXPRESSION CASSETTE. Applicant: グランドグリーン株式会社. The sequence listing filed with the application follows.

SEQUENCE LISTING (68 sequences)

SEQ ID NO: 1 - DNA, 459 bp, synthetic construct
  misc_feature 1..459: note = 1
  source 1..459: mol_type = other DNA
tggcagacatactgtcccacaaatgaagatggaatctgtaaaagaaaacgcgtgaaataatgcgtctgacaaaggttaggtcggctgcctttaatcaataccaaagtggtccctaccacgatggaaaaactgtgcagtcggtttggctttttctgacgaacaaataagattcgtggccgacaggtgggggtccaccatgtgaaggcatcttcagactccaataatggagcaatgacgtaagggcttacgaaataagtaagggtagtttgggaaatgtccactcacccgtcagtctataaatacttagcccctccctcattgttaagggagcaaaatctcagagagatagtcctagagagagaaagagagcaagtagcctagaagtagtcaaggcggcgaagtattcaggcaggtggccaggaagaagaaaagccaagacgacgaaaacaggtaagagct

SEQ ID NO: 2 - DNA, 181 bp, synthetic construct
  misc_feature 1..181: note = 2
  source 1..181: mol_type = other DNA
atgctccacaaagacgcactacagaagactaaagagagctttttcataccaaagaagtacaacaaagatttgctcctcattttctgaatcctgggactctctagcctgtagaagaagaaaggcaggaatttcagctcaagagaacagatcacaatatttacccacggcactgtctcgcaat

SEQ ID NO: 3 - DNA, 4272 bp, synthetic construct
  misc_feature 1..4101: note = 3
  source 1..4272: mol_type = other DNA
atggactataaggaccacgacggagactacaaggatcatgatattgattacaaagacgatgacgataagatggccccaaagaagaagcggaaggtcggtatccacggagtcccagcagccgacaagaagtacagcatcggcctggacatcggcaccaactctgtgggctgggccgtgatcaccgacgagtacaaggtgcccagcaagaaattcaaggtgctgggcaacaccgaccggcacagcatcaagaagaacctgatcggagccctgctgttcgacagcggcgaaacagccgaggccacccggctgaagagaaccgccagaagaagatacaccagacggaagaaccggatctgctatctgcaagagatcttcagcaacgagatggccaaggtggacgacagcttcttccacagactggaagagtccttcctggtggaagaggataagaagcacgagcggcaccccatcttcggcaacatcgtggacgaggtggcctaccacgagaagtaccccaccatctaccacctgagaaagaaactggtggacagcaccgacaaggccgacctgcggctgatctatctggccctggcccacatgatcaagttccggggccacttcctgatcgagggcgacctgaaccccgacaacagcgacgtggacaagctgttcatccagctggtgcagacctacaaccagctgttcgaggaaaaccccatcaacgccagcggcgtggacgccaaggccatcctgtctgccagactgagcaagagcagacggctggaaaatctgatcgcccagctgcccggcgagaagaagaatggcctgttcggaaacctgattgccctgagcctgggcctgacccccaacttcaagagcaacttcgacctggccgaggatgccaaactgcagctgagcaaggacacctacgacgacgacctggacaacctgctggcccagatcggcgaccagtacgccgacctgtttctggccgccaagaacctgtccgacgccatcctgctgagcgacatcctgagagtgaacaccgagatcaccaaggcccccctgagcgcctctatgatcaagagatacgacgagcaccaccaggacctgaccctgctgaaagctctcgtgcggcagcagctgcctgagaagtacaaagagattttcttcgaccagagcaagaacggctacgccggctacattgacggcggagccagccaggaagagttctacaagttcatcaagcccatcctggaaaagatggacggcaccgaggaactgctcgtgaagctgaacagagaggacctgctgcggaagcagcggaccttcgacaacggcagcatcccccaccagatccacctgggagagctgcacgccattctgcggcggcaggaagatttttacccattcctgaaggacaaccgggaaaagatcgagaagatcctgaccttccgcatcccctactacgtgggccctctggccaggggaaacagcagattcgcctggatgaccagaaagagcgaggaaaccatcaccccctggaacttcgaggaagtggtggacaagggcgcttccgcccagagcttcatcgagcggatgaccaacttcgataagaacctgcccaacgagaaggtgctgcccaagcacagcctgctgtacgagtacttcaccgtgtataacgagctgaccaaagtgaaatacgtgaccgagggaatgagaaagcccgccttcctgagcggcgagcagaaaaaggccatcgtggacctgctgttcaagaccaaccggaaagtgaccgtgaagcagctgaaagaggactacttcaagaaaatcgagtgcttcgactccgtggaaatctccggcgtggaagatcggttcaacgcctccctgggcacataccacgatctgctgaaaattatcaaggacaaggacttcctggacaatgaggaaaacgaggacattctggaagatatcgtgctgaccctgacactgtttgaggacagagagatgatcgaggaacggctgaaaacctatgcccacctgttcgacgacaaagtgatgaagcagctgaagcggcggagatacaccggctggggcaggctgagccggaagctgatcaacggcatccgggacaagcagtccggcaagacaatcctggatttcctgaagtccgacggcttcgccaacagaaacttcatgcagctgatccacgacgacagcctgacctttaaagaggacatccagaaagcccaggtgtccggccagggcgatagcctgcacgagcacattgccaatctggccggcagccccgccattaagaagggcatcctgcagacagtgaaggtggtggacgagctcgtgaaagtgatgggccggcacaagcccgagaacatcgtgatcgaaatggccagagagaaccagaccacccagaagggacagaagaacagccgcgagagaatgaagcggatcgaagagggcatcaaagagctgggcagccagatcctgaaagaacaccccgtggaaaacacccagctgcagaacgagaagctgtacctgtactacctgcagaatgggcgggatatgtacgtggaccaggaactggacatcaaccggctgtccgactacgatgtggaccatatcgtgcctcagagctttctgaaggacgactccatcgacaacaaggtgctgaccagaagcgacaagaaccggggcaagagcgacaacgtgccctccgaagaggtcgtgaagaagatgaagaactactggcggcagctgctgaacgccaagctgattacccagagaaagttcgacaatctgaccaaggccgagagaggcggcctgagcgaactggataaggccggcttcatcaagagacagctggtggaaacccggcagatcacaaagcacgtggcacagatcctggactcccggatgaacactaagtacgacgagaatgacaagctgatccgggaagtgaaagtgatcaccctgaagtccaagctggtgtccgatttccggaaggatttccagttttacaaagtgcgcgagatcaacaactaccaccacgcccacgacgcctacctgaacgccgtcgtgggaaccgccctgatcaaaaagtaccctaagctggaaagcgagttcgtgtacggcgactacaaggtgtacgacgtgcggaagatgatcgccaagagcgagcaggaaatcggcaaggctaccgccaagtacttcttctacagcaacatcatgaactttttcaagaccgagattaccctggccaacggcgagatccggaagcggcctctgatcgagacaaacggcgaaaccggggagatcgtgtgggataagggccgggattttgccaccgtgcggaaagtgctgagcatgccccaagtgaatatcgtgaaaaagaccgaggtgcagacaggcggcttcagcaaagagtctatcctgcccaagaggaacagcgataagctgatcgccagaaagaaggactgggaccctaagaagtacggcggcttcgacagccccaccgtggcctattctgtgctggtggtggccaaagtggaaaagggcaagtccaagaaactgaagagtgtgaaagagctgctggggatcaccatcatggaaagaagcagcttcgagaagaatcccatcgactttctggaagccaagggctacaaagaagtgaaaaaggacctgatcatcaagctgcctaagtactccctgttcgagctggaaaacggccggaagagaatgctggcctctgccggcgaactgcagaagggaaacgaactggccctgccctccaaatatgtgaacttcctgtacctggccagccactatgagaagctgaagggctcccccgaggataatgagcagaaacagctgtttgtggaacagcacaagcactacctggacgagatcatcgagcagatcagcgagttctccaagagagtgatcctggccgacgctaatctggacaaagtgctgtccgcctacaacaagcaccgggataagcccatcagagagcaggccgagaatatcatccacctgtttaccctgaccaatctgggagcccctgccgccttcaagtactttgacaccaccatcgaccggaagaggtacaccagcaccaaagaggtgctggacgccaccctgatccaccagagcatcaccggcctgtacgagacacggatcgacctgtctcagctgggaggcgacaaaaggccggcggccacgaaaaaggccggccaggcaaaaaagaaaaagtaa

SEQ ID NO: 4 - DNA, 211 bp, synthetic construct
  misc_feature 1..211: note = 4
  source 1..211: mol_type = other DNA
gtccgcaaaaatcaccagtctctctctacaaatctatctctctctatttttctccagaataatgtgtgagtagttcccagataagggaattagggttcttatagggtttcgctcatgtgttgagcatataagaaacccttagtatgtatttgtatttgtaaaatacttctatcaataaaatttctaattcctaaaaccaaaatccagtgac

SEQ ID NO: 5 - DNA, 1038 bp, synthetic construct
  misc_feature 1..1038: note = 5
  source 1..1038: mol_type = other DNA
atacagcattcccagaaagagaaacagaagaaatatacaaactttcattttgagagcagcacctcgtctattgattgcagataatatgcttctcatttgtatttccttttgattatttttgtttctatccctttgtttgagtcaatctcaaatattcggtcattgttggtatgaaaaatcaagcagttcatgttaagagtcaatttaaaattaatatttttatatagagttgtatgtgaaatgatgttgtgatttggtatatatggataaagagcttgtcagttcattttggtgtcatttttttggtatccaaataagaaacacaaaagggatatgtccctctactatcaaatattagttataagtattcatgttatactattcgatattttctaccccaatcgttacctatttaaaagtatttacccctccatctatcaaacccctggacccagctttcctattacatgtggcttcatcttaagcccccaaacctttttcttatttttgatttttaaaggctcatcttaaaatttattactcaaattaatacctcttaataacccacctcaaggacccagtaattaaatatccaattagctccagtaattggggttcatattagctccagtcttaaattttaaaggcgatgatcgtattcctccacttggttcatttatactcaaagaatactcaatgtctttagtgtttagataactttttgtaaatcatatagattgttttaacaaaaaacaattcaatagtagattttcacatgaaagttacataaaaattctttaaaattactttctcaaaaaattgttccaaacatattatcccacaattaaactcaatctgtttttcgaaacctaaatcaaaaccaatccaactaccttatataatatataatcaatacattgtaaagaactgcatgttcttttaaattttgggggcaaagttattccgtacgttcacacatgtactaataggaggtaataaatgatatgtgaaacaatcgaggtgtaaacaagctagcat

SEQ ID NO: 6 - DNA, 1169 bp, synthetic construct
  misc_feature 1..1169: note = 6
  source 1..1169: mol_type = other DNA
tcgattaaaaatcccaattatatttggtctaatttagtttggtattgagtaaaacaaattcgaaccaaaccaaaatataaatatatagtttttatatatatgcctttaagactttttatagaattttctttaaaaaatatctagaaatatttgcgactcttctggcatgtaatatttcgttaaatatgaagtgctccatttttattaactttaaataattggttgtacgatcactttcttatcaagtgttactaaaatgcgtcaatctctttgttcttccatattcatatgtcaaaatctatcaaaattcttatatatctttttcgaatttgaagtgaaatttcgataatttaaaattaaatagaacatatcattatttaggtatcatattgatttttatacttaattactaaatttggttaactttgaaagtgtacatcaacgaaaaattagtcaaacgactaaaataaataaatatcatgtgttattaagaaaattctcctataagaatattttaatagatcatatgtttgtaaaaaaaattaatttttactaacacatatatttacttatcaaaaatttgacaaagtaagattaaaataatattcatctaacaaaaaaaaaaccagaaaatgctgaaaacccggcaaaaccgaaccaatccaaaccgatatagttggtttggtttgattttgatataaaccgaaccaactcggtccatttgcacccctaatcataatagctttaatatttcaagatattattaagttaacgttgtcaatatcctggaaattttgcaaaatgaatcaagcctatatggctgtaatatgaatttaaaagcagctcgatgtggtggtaatatgtaatttacttgattctaaaaaaatatcccaagtattaataatttctgctaggaagaaggttagctacgatttacagcaaagccagaatacaaagaaccataaagtgattgaagctcgaaatatacgaaggaacaaatatttttaaaaaaatacgcaatgacttggaacaaaagaaagtgatatattttttgttcttaaacaagcatcccctctaaagaatggcagttttcctttgcatgtaactattatgctcccttcgttacaaaaattttggactactattgggaacttcttctgaaaatagtg

SEQ ID NO: 7 - DNA, 450 bp, synthetic construct
  misc_feature 1..443: note = 7
  source 1..450: mol_type = other DNA
cctgcatcgttgaacaacggaaactcgacttgccttccgcacaatacatcatttcttcttagctttttttcttcttcttcgttcatacagtttttttttgtttatcagcttacattttcttgaaccgtagctttcgttttcttctttttaactttccattcggagtttttgtatcttgtttcatagtttgtcccaggattagaatgattaggcatcgaaccttcaagaatttgattgaataaaacatcttcattcttaagatatgaagataatcttcaaaaggcccctgggaatctgaaagaagagaagcaggcccatttatatgggaaagaacaatagtatttcttatataggcccatttaagttgaaaacaatcttcaaaagtcccacatcgcttagataagaaaacgaagctgagtttatatacagctagagtcgaagtagtgattg

SEQ ID NO: 8 - DNA, 109 bp, synthetic construct
  misc_feature 1..21: note = 8
  source 1..109: mol_type = other DNA
gttggtagtagcgactccatggttttagagctagaaatagcaagttaaaataaggctagtccgttatcaacttgaaaaagtggcaccgagtcggtgctttttttttttt

SEQ ID NO: 9 - DNA, 262 bp, synthetic construct
  misc_feature 1..262: note = 9
  source 1..262: mol_type = other DNA
ccggctgcagatcgttcaaacatttggcaataaagtttcttaagattgaatcctgttgccggtcttgcgatgattatcatataatttctgttgaattacgttaagcatgtaataattaacatgtaatgcatgacgttatttatgagatgggtttttatgattagagtcccgcaattatacatttaatacgcgatagaaaacaaaatatagcgcgcaaactaggataaattatcgcgcgcggtgtcatctatgttactagatc

SEQ ID NO: 10 - DNA, 909 bp, synthetic construct
  misc_feature 1..909: note = 10
  source 1..909: mol_type = other DNA
atggcagctaacgcaggaggaggaggagcaggaggtggatcaggttcaggaagtgtggcagcaccagcagtttgtagaccaagtggatctagatggactccaacacctgaacaaatcagaatgcttaaggagttgtactacggttgtggaatcagatcaccttcttcagaacagattcaaagaattactgctatgcttagacagcatggaaaaattgaaggaaaaaatgttttctattggttccaaaaccataaggctagagagagacagaaaagaagattgacttctcttgatgttaatgttcctgctgctggtgctgctgatgctactacatctcaacttggagttctttcactttcttctcctcctccttctggtgctgctccaccttcaccaactttgggtttttatgctgctggaaatggtggaggatctgctgttcttttggatacatcttcagattggggttcttcaggagctgctatggctactgaaacatgttttcttcaagattacatgggtgttactgatacaggatcttcatctcagtggccaagattctcatcttcagatactattatggctgctgctgctgctagagctgctactacaagagctcctgagactcttccattgtttcctacatgtggagatgatggtggatctggatcttcatcttatttgccattctggggtgctgcttcaactacagctggagctacttcatctgttgctattcaacagcaacatcagcttcaagagcagtactctttctattcaaactctaactcaactcaattggctggtacaggaaatcaggatgtttcagctacagctgctgctgctgctgctttagagttgtcattatcaagttggtgtagtccttatccagcagcaggtagtatgtga

SEQ ID NO: 11 - protein, 302 aa, synthetic construct
  REGION 1..302: note = 11
MAANAGGGGAGGGSGSGSVAAPAVCRPSGSRWTPTPEQIRMLKELYYGCGIRSPSSEQIQRITAMLRQHGKIEGKNVFYWFQNHKARERQKRRLTSLDVNVPAAGAADATTSQLGVLSLSSPPPSGAAPPSPTLGFYAAGNGGGSAVLLDTSSDWGSSGAAMATETCFLQDYMGVTDTGSSSQWPRFSSSDTIMAAAAARAATTRAPETLPLFPTCGDDGGSGSSSYLPFWGAASTTAGATSSVAIQQQHQLQEQYSFYSNSNSTQLAGTGNQDVSATAAAAAALELSLSSWCSPYPAAGSM

SEQ ID NO: 12 - DNA, 723 bp, synthetic construct
  misc_feature 1..723: note = 12
  source 1..723: mol_type = other DNA
atggatctgcgtctaattttcggtccaacttgcacaggaaagacgtcgaccgcgatacgtcttgcccagcagactggccttccagtcctttcgctcgatcgggtccaatgctgtcctcaactgtcaaccggaagcggacgaccaacagtggaagaactgaaaggaacgacccgtctataccttgaagatcggcctctggtgaagggtatcatcgcagccaagcaagctcacgaaaggctgatcggggaagtgtacaattatgaggcccacggcgggcttattcttgagggaggatctatctcgttgctcaggtgcatggcgcaaagcagttattggagtaccgattttcgttggcatattattcgccacaagttagcagacgaggagacattcatgaacgcggccaaggccagagttaggcagatgttgcgccctgctgtaggcccatctattattcaagagttggttcatctttggaatgagcctcggctgaggcccatactgaaagagatcgacggatatcgatatgccatgttatttgctagccagaaccagatcacacccgatatgctattgcagcttgacccagatatggagggtgagttgattcatggaatcgctcaggagtatctcatccatgcgcgccggcaggagcaggaattccctccagtgagcgtggtcgctttcgaaggattcgaaggtccaccgttcggaatgtgctag

SEQ ID NO: 13 - protein, 240 aa, synthetic construct
  REGION 1..240: note = 13
MDLRLIFGPTCTGKTSTAIRLAQQTGLPVLSLDRVQCCPQLSTGSGRPTVEELKGTTRLYLEDRPLVKGIIAAKQAHERLIGEVYNYEAHGGLILEGGSISLLRCMAQSSYWSTDFRWHIIRHKLADEETFMNAAKARVRQMLRPAVGPSIIQELVHLWNEPRLRPILKEIDGYRYAMLFASQNQITPDMLLQLDPDMEGELIHGIAQEYLIHARRQEQEFPPVSVVAFEGFEGPPFGMC

SEQ ID NO: 14 - DNA, 306 bp, synthetic construct
  misc_feature 1..306: note = 14
  source 1..306: mol_type = other DNA
gaaaagcagaatgctgagctaaaagaaaggctttttccattttcgagagacaatgagaaaagaagaagaagaagaagaagaagaagaagaagaaaagagtaaataataaagccccacaggaggcgaagttcttgtagctccatgttatctaagttattgatattgtttgccctatattttatttctgtcattgtgtatgttttgttcagtttcgatctccttgcaaaatgcagagattatgagatgaataaactaagttatattattatacgtgttaatattctcctcctctctctagctagcctt

SEQ ID NO: 15 - DNA, 431 bp, synthetic construct
  misc_feature 1..431: note = 15
  source 1..431: mol_type = other DNA
gttgttggttggcacaccacaaatatactgttgccgagcacaattgatcggctaaatggtatggcaagaaaaggtatgcaatataataatcttttattgggtatgcaacgaaaatttgtttcgtcaacgtatgcaatattctttattaaaagagggtatgcaatgtattttattaaaaacgggtatgcaatataataatcttttattgggtatgcaacgaaaatttgtttcgtcaaagtatgcaatattttttattaaaagagggtatgcaatgtattttattaaaaacgggtatgcaataaaaaattatttggtttctctaaaaagtatgcagcacttattttttgataaggtatgcaacaaaattttactttgccgaaaatatgcaatgtttttgcgaataaattcaacgcacacttattacgtggcca

SEQ ID NO: 16 - DNA, 1971 bp, synthetic construct
  misc_feature 1..1971: note = 16
  source 1..1971: mol_type = other DNA
gaattccagaaatctttgatttcagatgcttgagggagtgtcctgatcctaagtgcttcttgcacttcaccagcttgactttccatctctcactgggcccactgcagcacacacttggctccagctggaaaatcctgaacagagcttcccggcaggtgaactgccataagtgggttataagcttgctgagatagtgttcagagtgcccatgtacctggggtggctggagcccctgagccagcccctcccagtcaggagcactacaaatacagttttccatgtaagccatcaatatgacaacagttgggaggcactgctgtgaaaaacagaacactgactaactcactccccaaaatgcaggagtgttcctaggagtatttctagaaggtccttcatttccctttttccctacatccacttcatcagtaagacctgtcagttctaccatgaaaatatatctccaatccatctacttcttccatctccactgcaaccaccttctataaacaccatcatctcttacagggactgcttcaataacccactaactggcccccttgcttctgctcttgtccctggacaatccattctccagttcttcataaaatgtacatcagatgatgacagctggacctccttcccaggcctgtaacatctgcaaacgatctggcccttgcttcctccccagcctcacctcacatctgctccttctctttcttcccttcagctgcagtggccttccttctcgtcctttctatgtctctcttttctagctacctgaaactctgtctccaatttttcacagttctcagctccaactaaattagtcacccatgccacccataaccaacctcaattacatctctgttcttattttccctcacatcactatctgaaatcatcagattcatacatgtttattttatgtctctcccatctcacctctcccctacacacacacacacacacacacacacacacacacacacacacacacacgataatataaactatatgagggcagggagcttatcttttcactgatatgtctccagcccctgggcttgtgttgaccgcatcacagacaatcagtaaatatctgtgtaaaaaaaaggaatgcaatttcttcacttaaaaactcaccattcacctagatttaggaaataaaaatacaagacacccagttaaatgtgcatttcaaataaacaacaaaaatttcagtaatacgggtagctgggacatgccatatttggaacacatttatactaaaaaagtattcattgtttatctgaaattcaaattccactgggcatcctgtgttttatctggcaatgctaggcatgcagaataccaaaagtaagcaccaggcaggccagagtcccaccatgagcatcttcagggcccctggatgtggaagagggatgttgagggcccaggggctgccttgccggtgcattggctgcccaggcctgcactgccgcctgccggcaggggtccagtccacgagacgcagctccctgctggcggaagtccatttcagagcttccggttctcccaagtccaaggattatgctcactccccacccacagtctcttagtgtctgtccctgctctaaagatgttgtctgggcttgatattaatatgagagctgactgttcccttcctgatctagaccataaccatcttcaagttaaattgctcctcctcttctaactgcccaacctcacccacgtctgaccatacccaagcacagagaagtgggtttaatggaccttcacacagaaggacacatcctctcctataatgctttacatggaaggttcagacataacctgagtcctgcttggggtagcatcatcatgactctcttgccctggtgtccttgcaatattccttgaaaggcatccctcccccaaggaagggcaggcactgagcacagcaatgcagtataatggctaagagtgggatcc

SEQ ID NO: 17 - DNA, 574 bp, synthetic construct
  misc_feature 1..574: note = 17
  source 1..574: mol_type = other DNA
cccgggagcagaacccctgtaagctcaggggtttttaggcgtttaattacggtcagatgagcaatttttgataccttaatttgttgtgacactggtagttaactattcattctttcttgctctcttgctttctatttctctttaaaatgcttttccaaaagaatggggggggggggctggacgctcccgaaccccgacgttccgcgggccctgacatgtaagcatctcaagaagcatatttcttgcctggctgttaatttacaaacgcataaaaaaaatataatttactaaagaatgaggaaaaatctcgggaagttatgtaatttcagcattatgtgtaaaccaccgttatggaataagaaataaaccacatttcaatttatttcccccgagcccccctccccgatcaatacgccagtgccccgccccgcccgcctcccgatctacactttgttggcggaaaaaatcgcaactgatctcccctacctttcttctttctctttcccttgctctcctcttaccctttcccttccccacccttctccacaacttgttggcgggattacctgcaaat

SEQ ID NO: 18 - DNA, 284 bp, synthetic construct
  misc_feature 1..284: note = 18
  source 1..284: mol_type = other DNA
gccatcaagcttgcctcgtcccgccgggtcacccggccagcgacatggaggcccagaataccctccttgacagtcttgacgtgcgcagctcaggggcatgatgtgactgtcgcccgtacatttagcccatacatccccatgtataatcatttgcatccatacattttgatggccgcacggcgcgaacgaaaaattacggctcctcgctgcagacctgcgagcagggaaacgctcccctcacagacgcgttgaattctccccacggcgcgcccctgtagagaaat

SEQ ID NO: 19 - DNA, 526 bp, synthetic construct
  misc_feature 1..526: note = 19
  source 1..526: mol_type = other DNA
ccgtatacttacatatagtagatgtcaagcgtaggcgcttcccctgccggctgtgagggcgccataaccaaggtatctatagaccgccaatcagcaaactacctccgtacattcatgttgcacccacacatttatacacccagaccgcgacaaattacccataaggttgtttgtgacggcgtcgtacaagagaacgtgggaactttttaggctcaccaaaaaagaaagaaaaaatacgagttgctgacagaagcctcaagaaaaaaaaaattcttcttcgactatgctggaggcagagatgatcgagccggtagttaactatatatagctaaattggttccatcaccttcttttctggtgtcgctccttctagtgctatttctggcttttcctatttttttttttccatttttctttctctctttctaatatataaattctcttgcattttctatttttctctctatctattctacttgtttattcccttcaaggtttttttttaaggagtacttgtttttagaat

SEQ ID NO: 20 - DNA, 459 bp, synthetic construct; identical to SEQ ID NO: 1
  misc_feature 1..459: note = 20
  source 1..459: mol_type = other DNA

SEQ ID NO: 21 - DNA, 1908 bp, synthetic construct
  misc_feature 1..1908: note = 21
  source 1..1908: mol_type = other DNA
gaaacaagtgtccgaaatcctacttcggtttttcagagacctctctaaagtgatatattcccgacaaaatggttattttacaaaaaaaataatcattttttttcaaattattcatttatatgggttagaatactcaatttccctgtgttatttaatttaaaatcatttccaatatacaaacatactttattatctgattatttataataaattttcataaagtttcacctaatcttttattccttatattataaaatttatccatccaaatcaaacttattttgtataatttaaaagtattttcaatataatcatttggtttgtggtgacgtagtaaaacatatgaaatatatgatgtataacttattgatcaatgttcaaattttgacactactcggtcctgtggccataaatgtttgtcggcattgactccaaaacatgaagtatcctctttaataaattaaagtttttttttgtcacttgtcacactctcatgcattatacaaaatgtcattttgtcataattttgagatatttatttttcatttgtcatttacttcactttttatttttgaatatatccttaatttagtttttataaattaaccatatcataataactatattaattttaaattttgaatttcaaacttcaatcgaaactttaaataaatttacaattgaaacgtttgtatttaacattttgttataattagacatttgatacacgagtcagataactaaacacataattttaatttatttttttcattttttttttataattcttacttattccaaatttcaaattcaaataaatttgctgtttaatcattcgtatttaacattttattgtaatcaacccgtataatatacaagtatcacaactactaacctcatatttgcagcgaaagattattcggcgtgcaaaagcagggcaaaaaaacccttgttagaaagtttcttttccaaaataaaaaattaaaaaataaaagtattttcaatatcaataacatactctattctctaattatttattactaacttttcaaagagattaacctaatcttgtattccttaaattataaaatttacaaattatatggatccaaaaccaaatatcccatcgactcaagatttaagttaaaagtttcttggacgaaacacaaagaaaagatattatcctaacccaaaagaagacggcagccttagaaatcaccgccactgattaaatatcggaatccaacgactctaatttcagacccttcatcaactttttattgacacgtgtcatattttcgtccgtttgtatctaacaacccgtagcgttagccttccttttcgtgaagaaaccttttcttatcctataaatccacccccaaatccatcgtcttccttcatcctgcaatcatctttatcttcaaagctctgacttcttcaattctcccaaggtattatcttttttattcttttatgtttgtttagtttttgaacagtttattttcaatcgattaaaggttattattgtttttgatctgtttgtggcttttgatttaagatataacctgatgttgtaattaacacgattgatagtgtcttaatatgttttaattatggtttctagatctaatcatcgaatttattaacgatctgttatagtttcgtgttttcgatcgtttttcaacaagtcaattccaaaatcgatgttattgtataaaagcttcgaacgacgattttttgtaaattaattcacgatctaagttttcaatttcagagaataaagttgttgatttgtttttgaattgtaatctgatctctgtttcaagtacgatatgaatttgtttgttgatgaattgatgataaaactgttttcgttttctaataattgtttcgttctttttttaacag

SEQ ID NO: 22 - DNA, 2432 bp, synthetic construct
  misc_feature 1..2432: note = 22
  source 1..2432: mol_type = other DNA
acataagtctatctaaaatggaaagattgttacctaatctcaaatcatatttttcccatcataaaaaaaaatctcaaatcatgtgatcttgtcgatcatcatttaatacattattaattcttctttttaattgaaaaatgtgattatatgttatgtggagattagttcagaccatgatccttgaatatgtagtaagtttttgtaatgttgagtttgagttctttgacactaggtccatgtttcccaaaattaagtgtaaaaaataaataaagaattaaaagttgtgaaaaaaattgtcctcgtttatttttattattcagaattaatctttattgagactaaaattatttacagaaagttaatacagcactaaaagttattttatttttttgagaaacaaaaactgaaatctaaaaaaaaataagaaaccggaaatctaattaacaaaaatatatacgggctaacatggttatgggcttaggctgcctcattacccattacatgctctgttcctaaaaaaaaaaagaagtttgggcctttatcctccagtaagttttttaattgggctcaagaactttaggatttaggtgaggatcaatgaaagtttatatattaggcttgatttttttttcaatttacgtaaaaatgaaagaaaaagtcacactctataaactttatttttttcaatattaatacattgttattgtggatatatcattagcggaaaagtaattctaataccagatttaattgactttgactaatttttttagcggaataaaagttttgttactttgtcgcgtgatttttaatcaaactttggggataatttcccctccaattcagcccaaaaaaaaaaaaaactgacaccatatattattagtaggcaacttgttcgtaaatggtgtggcttatccgaatggaaattggattcgttttctttaacatcattattgtttttgtcaatgagctatcttttagtcttatgttattggtgaatctgtccttaagttgcatcatttaacacatctcctcattagagaaaaaaattcttccctaaacgattggtagtaaaaacatctaataagaaataagaaagaaaaattaggaaaaaggaaagttcattaaaaaaaatattttgaattattttttaaaaaatatctaaatattttttaaatgaataattttatataaactgtaactaaatgtatacaagtaatgtatgttaaaaaaatacttgaaaaatctactgaaaatatatcttacaaggtgaaattaaataagaaagaatttagtggaataattatgattttatttaaaaaataattattaaagatttttttgctccataataagaaaacttttcaattattcttttctggtccataataaaaaaaatctagcatgacagcttttccatagatttttaataatgtaaaagcagccgacttcaggcaatggatagtggggcccgtatcaacttcggacgctccacttgcaacggggtgggcccaatataacaacgacgtcgtaacagataaagcgaagcttgaaggtgcatgtgactccgtcaagattacgaaaccgccaactaccacgcaaattgcaattctcaatttcctagaaggactctccgaaaatgcatccaataccaaatattacccgtgtcataggcaccaagtgacaccatacatgaacacgcgtcacaatatgactggagaagggttccacaccttatgctataaaacgccccacacccctcctccttccttcgcagttcaattccaatatattccattctctctgtgtatttccctacctctcccttcaaggttagtcgatttcttctgtttttcttcttcgttctttccatgaattgtgtatgttctttgatcaatacgatgttgatttgattgtgttttgtttggtttcatcgatcttcaattttcataatcagattcagcttttattatctttacaacaacgtccttaatttgatgattctttaatcgtagatttgctctaattagagctttttcatgtcagatccctttacaacaagccttaattgttgattcattaatcgtagattagggcttttttcattgattacttcagatccgttaaacgtaaccatagatcagggctttttcatgaattacttcagatccgttaaacaacagccttattttttatacttctgtggtttttcaagaaattgttcagatccgttgacaaaaagccttattcgttgattctatatcgtttttcgagagatattgctcagatctgttagcaactgccttgtttgttgattctattgccgtggattagggttttttttcacgagattgcttcagatccgtacttaagattacgtaatggattttgattctgatttatctgtgattgttgactcgacaggatccatg

SEQ ID NO: 23 - DNA, 1616 bp, synthetic construct
  misc_feature 1..1616: note = 23
  source 1..1616: mol_type = other DNA
tcatatcaaacacgtcctccatggctatcagaccgatcacaaggttctctacctcctcctcagtattctcgatacgctcgagtggaatctcatcaataaagtttagtatcgcgtcgatacgatcctcatacctgaccaatttagcagcaagcaaaggaatggtgtgatggcgcaattaaattaacccgataagcattttcaacccgattaaacccgacccgataagccttatcgtgttcgggtcgggttaacccgaccctattgacacccctagtgtcaagtataaacattttcaagtaattaacccaaatacaaaatacataacactagttatttaacatgcaaattactatatagtttagggtgtaaggtgttataaatttatttacaaggacctaaagtggtaggttaaatgttaaattagcaaattacttattttatgcaaatcatcttataaataccaattttcatcaaccattattcagtcgagaaactaattaacatcgagagattagcagcggttttttttgccagagaattaaggtaacatgcaaacctgtggttattaatttaatttttgaatttttattcaatggatgttaagtttctgaggcaatatgtggaggataacccaaattggttggaaatcgaggggattttttttgtgaagtgagttcgtaattatttatttgttaagttttcctattgattcattggtgttttaagctaataccagtgaagtaatattgataatccatttatgttgttgagttaagagatagttaatttatgatatatatctcgataactctgagttagtaattgcctatgctatgctgctgaatcattgtgttctatctcttctcgaacgatgtctgttatacacttgtcgatcatatgcttcatttattttgtaacattttttatcaacttcgggtgactttcgtgtgaatagatactctaagatgcgattaaatcataatcaagatgttaataaatccctttttccttaaaatatctttttttgtgactaataataccttgtacatatttatatgcttgcagactaactatcaataaccgtcatggataattaccatgatgaaaacgacatctttgatgggaaatcgggccgtaatagacccactctctttcttggaggcattggaccgatgcagatatggattgagaccctcatcggtgtgaccatgactcttaaagttgagagctccagcaccattggcgacattgtaaccatgatcagagacaagttagggattccccgatatctctcgcatacgatcttggttcacggagagaaggtcatcaatggaaaatcttctgttgatgattgccacatcgagatgggatccactctgttgttctttgtggcacggatgcaggagatattggctgaaaggcggcaggagggagttgttcttgttcaagaccatcaccagagacggcttttatttactcaaaagcagctcattctgcaaaagttatttataataaaatgggatgatggaaaaaccttggctctagaagtcaaaacctccgacaccatcatcgatgtgagaattcagatccaacgtgagctacatattcctctatgc

SEQ ID NO: 24 - DNA, 1618 bp, synthetic construct
  misc_feature 1..1618: note = 24
  source 1..1618: mol_type = other DNA
tcatatcaaacacgtcctccatggctatcagaccgatcacaaggttctctacctcctcctcagtattctcgatacgctcgagtggaatctcatcaataaagtttaggatcgcgtcgatacgatcctcatacctgaccaatttagcagctagcaaaggaatggtgtgatggcgcaattaaattaacccgataaacattttcaacccgatttaccccgacccgataagccttatcgggttcgggtcgggtcaacctgaccctattgacacccctagtgtcaagtataaacattttcaagtaattaacccaaatacaaaatacataacactagttatttaacatgcaaattactatatagtttagggtgtaaggtgttataaatttatttacaaggacctaaagtggtaggttaaatgttaaattagcaaattacttattttatgcaaatcatcttataaataccaattttcatcaaccattattcagtcgagaaactaattaacatcgagagattagcagcggtttttttgcgagagaattaaggtaacatgcaaacctgtggttattaatttaatttttgaatttttattcaatggatgttaagtttatgaggcaatatgtggaggataacccaaattggttggaaatcgaggggattttttttgtgaagtgagttcgtaattacttatttgttaagttttcctattgattcattggtgttttaagctaataccagagaagtaatattgataatccatttatgttgttgagtaaagagatagttactttatgataaatatatcgataaatctgagttagtaattgcctatgctatgctgctgaatcattgtggtgtatcgctacttatacgatggtctgttatacgcttgtcgatcatatgcttcatttatttagtaaatttttttttatcaacttcgggtgactttcgtgtgaatatatactctaagatgcgattaaatcataatcaagatgttaataaatccctttttccttaaaatatctttttttgtgactaataataccttgtacatatttatatgcttgcagactaactatcaataaccgtcatggataattaccatgatgaaaacgacatctttgatgggaagtcgggccgtaatagacccactctctttcttggaggcattggaccgatgcagatatggattgagaccctcatcggtgtgaccatgactcttaaagttgagagctccagcaccattggcgacattgtaaccatgatcagagacaagttagggattccccaatatctcccgcatacgatcttggttcacggagaggaggtcatcaatggaaaatcttctgttgatgattgccacatcgagatgggatccactctgttgttctttgtggcacggatgcaggagatattggctgaaaggcggcaggagggagttgttcttgttcaagaccatcaccagagacggcgtttatttactcaaaggcagttcgttctgcaaaagttatttataataaaatgggatgatggaaagaccttggctctagaagtcaaaacctccaacaccatcatcgatgtgagaattcagatccaacgtgagctacatattcctctatgc

SEQ ID NO: 25 - DNA, 1618 bp, synthetic construct
  misc_feature 1..1618: note = 25
  source 1..1618: mol_type = other DNA
tcatatcaaacacgtcctccatggctatcagaccgatcacaaggttctctacctcctcctcagtattctcgatacgctcgagtggaatctcatcaataaagtttaggatcgcgtcgatacgatcctcatacctgaccaatttagcagctagcaaaggaatggtgtgatggcgcaattaaattaacccgataaacattttcaacccgatttaccccgacccgataagccttatcgggttcgggtcgggtcaacctgaccctattgacacccctagtgtcaagtataaacattttcaagtaattaacccaaatacaaaatacataacactagttatttaacatgcaaattactatatagtttagggtgtaaggtgttataaatttatttacaaggacctaaagtggtaggttaaatgttaaattagcaaattacttattttatgcaaatcatcttataaataccaattttcatcaaccattattcagtcgagaaactaattaacatcgagagattagcagcggtttttttgcgagagaattaaggtaacatgcaaacctgtggttattaatttaatttttgaatttttattcaatggatgttaagtttatgaggcaatatgtggaggataacccaaattggttggaaatcgaggggattttttttgtgaagtgagttcgtaattacttatttgttaagttttcctattgattcattggtgttttaagctaataccagagaagtaatattgataatccatttatgttgttgagtaaagagatagttactttatgataaatatatcgataaatctgagttagtaattgcctatgctatgctgctgaatcattgtggtgtatcgctacttatacgatggtctgttatacgcttgtcgatcatatgcttcatttatttagtaaatttttttttatcaacttcgggtgactttcgtgtgaatatatactctaagatgcgattaaatcataatcaagatgttaataaatccctttttccttaaaatatctttttttgtgactaataataccttgtacatatttatatgcttgcagactaactatcaataaccgtcatggataattaccatgatgaaaacgacatctttgatgggaagtcgggccgtaatagacccactctctttcttggaggcattggaccgatgcagatatggattgagaccctcatcggtgtgaccatgactcttaaagttgagagctccagcaccattggcgacattgtaaccatgatcagagacaagttagggattccccaatatctcccgcatacgatcttggttcacggagaggaggtcatcaatggaaaatcttctgttgatgattgccacatcgagatgggatccactctgttgttctttgtggcacggatgcaggagatattggctgaaaggcggcaggagggagttgttcttgttcaagaccatcaccagagacggcttttatttactcaaaagcagctcattctgcaaaagttatttataataaaatgggatgatggaaaaaccttggctctagaagtcaaaacctccgacaccatcatcgatgtgagaattcagatccaacgtgagctacatattcctctatgc

SEQ ID NO: 26 - DNA, 972 bp, synthetic construct
  misc_feature 1..972: note = 26
  source 1..972: mol_type = other DNA
aaaaattacggatatgaatataggcatatccgtatccgaattatccgtttgacagctagcaacgattgtacaattgcttctttaaaaaaggaagaaagaaagaaagaaaagaatcaacatcagcgttaacaaacggccccgttacggcccaaacggtcatatagagtaacggcgttaagcgttgaaagactcctatcgaaatacgtaaccgcaaacgtgtcatagtcagatcccctcttccttcaccgcctcaaacacaaaaataatcttctacagcctatatatacaacccccccttctatctctcctttctcacaattcatcatctttctttctctacccccaattttaagaaatcctctcttctcctcttcattttcaaggtaaatctctctctctctctctctctctgttattccttgttttaattaggtatgtattattgctagtttgttaatctgcttatcttatgtatgccttatgtgaatatctttatcttgttcatctcatccgtttagaagctataaatttgttgatttgactgtgtatctacacgtggttatgtttatatctaatcagatatgaatttcttcatattgttgcgtttgtgtgtaccaatccgaaatcgttgatttttttcatttaatcgtgtagctaattgtacgtatacatatggatctacgtatcaattgttcatctgtttgtgtttgtatgtatacagatctgaaaacatcacttctctcatctgattgtgttgttacatacatagatatagatctgttatatcattttttttattaattgtgtatatatatatgtgcatagatctggattacatgattgtgattatttacatgattttgttatttacgtatgtatatatgtagatctggactttttggagttgttgacttgattgtatttgtgtgtgtatatgtgtgttctgatcttgatatgttatgtatgtgcagc

SEQ ID NO: 27 - DNA, 2195 bp, synthetic construct
  misc_feature 1..2195: note = 27
  source 1..2195: mol_type = other DNA
ttggttagatgatgccgaggatgattattactccttccgtttctatataaattcataaattaatcaaattacctaatccaccattgtatgaatacattaaatgagttaaatatagatgtttgaatgtattaaatgagggcaaatgtatgaaaaatatgaattttttgtctcgaatttgtagaatgatacttttttaaaacaaaattaaaatgatagaatgacacttattcagaaacgaagagagtattacataattttgcaattactaatccctttctaatttgaataaatatttaattataatttatcaatgatcttccatatctttaaataggaaaaatttcatattattccccggtgttttctcgaaaaaaaaaaatccttgtggtaaataaataatttaaaacccccatttgttatgtatgattaatcgtgaattatagttgctaaaaagagtgtacgattcttatttttacaagttttgtagtatttttttaaaatataatcaattttttaaaatagtagtttactaaatactgtaatttttaaataatataaaatatatttatatgtaataaaaatacgaaacttaggaaattatcaaaatagctaaaaattagtaatataactaaatactataatttttatgttatccttttattttattttatgcatttttttatgtttttatttcatgtacttttatctatttagtattttatatagttttattgtaggtgtaattttatctatttcagtattttttattgttggcctaatttttatctaatttatttttatgttttaacatttgaatttaattaaatttatcatatataataaattttaatattaattacaacacgttatttaaaatataaaacaaataacaaaagcaacatatacaaaataaaaataaaacactaaataataaacaataaataaagaaattgaaaaaaataaattaaattttttgaggtttgctacagctctcccctaaaatgcagtcgcagatggcatcccattacagaagtaagcaacagtattttgatgatttggcttggagacgcccatatagaatccacaagtagattcatataattattatgaataattcaacttataaattgccacattgttcatcaagtaacttcatatctattgttcaaaaaaaaaaaaaaaactttatatcaatatattccatgtgtggtttactattttttttttatatgaaaaaaacttccttcagttacctattcaaagacaagacagagaggaatacatattttcagtttaatcccgagaaatataaaatataaaatatttatgtagataataatgtaacaataaaaataaaagaaaatgaaaagagaaaaaagcgttggacgattaaagagagcgcgtggagcggtagccctcacgctgtcctgattatctccgccactcaaaaaggaacagatcaacttgcaattgccgtaaggaacctgtgcggtatacgtcattctgacacgtgtccttattttattggctactgcacgaggctgtttcctccttaagtcggcaacttctcctatataaaccacccccagttcgctttcaccctcattcgttaccagctacagatctaaccagctcattctttcttcttgttatcttctcgttctacgattttcttccttccctttcgtcaaggtacgaatttcttgtttttcgttgcttctctgtcgattatgcgttgatctgttttatttattattatgttgccgtctagagatctagcttttttttttttaattttaatgtctgccctctaattatctgtttatggttttcgttctcttagaattggttagatttttaattggatttgtatatttctaaatcccaattggtttatttctgttgtttaccgtgatttttcttaaatcccttcttttttatccgatctgtcgatcgctgtgattgacgcgattctttttttctttttttttgcttggccgaaataaaggctgctaatttattatttgtgcatcttgatttgttaatttctggatttgagtcgttatgaatagtttcgaaaatttagggtttgctattgattggtgttggatgttttcttgtgatttgattgaagtatagacgttatcgttcttgttcctgggaacttttattctgattcgttttcgacaatacag

SEQ ID NO: 28 - DNA, 2471 bp, synthetic construct
  misc_feature 1..2471: note = 28
  source 1..2471: mol_type = other DNA
aagattaattaggagccataaatacaggagttattttagggtacaattcatttaatatagatttgagccttaatgaaggcgttattttaggaggcaacatctggaaagattccgtttggtacatattgtgtaacaaaaacatgggatatgagagtaataaacaaacaatgcacaataatagtagtaaggtttgttatatgagatgtataggtaaaaatccctagaatataatgctaggacgcaaagttttggcttggaggccaatgatcaattgcgcttgagaggtgatgctgtaagggtcaatagtcatcttatttatactccatttcattcggtttaccataagtgtttaatttacctttttatttttgttcaaaataagtatttatttataaaatcaagaaagaattcaattttttttacaaaataacctttatgtatatatctctaaaaagttttcttacttctcacattaaatgtttaagtaaaggtagtttagtcataatagatatttttatataaaatttaatatttttttaatatgcgtgttaaaaacaaattaaacacttattgtgaaccggaggaagtaacacaagtatctcattggtggatggctaatgggacggtcggtgaacaaaaagcaaataaaacagcttcctcattgtgtttgccgttacatttcaaacgttatgaaaatacaattcaatatatatatatatatgtatatatatatatatattgcaaacaattgaattggttcaattgcatgataccaacgaatcaagtattaatttttattttttagaattaacctattgacgtggtgaaattattttagtaaaatttaattttttcaatttctgacaaccaaactgaataattgagttctttttgaatttccttcttgataaataacaactgcagtattaccaccatatggtattatgatgtatattatatatgcataaaaatatatggacaaacagaatgtataagccaacaaagtatgctctaaattttttttaaaaaaagttattcttttggaaaaaataaaaagaaccagaattatatgacatcggagcggatggagtaatacaaaagtatgtatgtaaatatttgtttagtggtctagaaaatgtgataataatatttaagaatatgatcaatgaaatcaatacattgaaagaataatcaaaaagtcttaggttaaagaatctcaacaaagataaaaaaaatttgatgatttgtttcatttggttgaataatagtaggcaaattaaaaatatgtggtaaaataaaaaataaaaatgtggaaacaaaaaactaggacgccgccgttgatgattaggtacaagaaagaaaaaagatctgaggggtaattaggtaaaccgactaaagtgcggcactaagagaagccctagctcatccttcgcctataaatagaccccaataaccccctgaaaccctaatcctctcatatattttcgtttctctctgtgctgtgcggcaacagatctatatttgctttcaaggttagatctaatcctctttcgtttctccgcagtttctatagacgtgttatttgctttgattaatctgattcattcatatctgtttgatgaaatcttcatatgtatgtctatacaattgctatttttatttaaaaaaagtatgcatgttgtatgattggtagactgtgctttctttgagtttgatgtgttagcattatcagattctataaatcattgattagctagtaagtttttattttcagtaagctgttttggttcattttttcaccataaatctcacgataattgaaattgcttgatagactttataatcggcttgattttgatagttattagtaatatctgtctagatttgtcgtgctttgctgtgcacgtatgatatgatacatggattaaagagttactgacgcctgatgtttacccatccaatgacatatgacgtgtgtcaacacatacactctttttcgctaatctgtggttaataactacacatgtttaccttaatttattactcaattccataaatttgatatggaatgaacactgggtatgggtagcagtaatcacatgtttactttaatgaccacacaaaacagatatcatagtttttatagttgaaaatattttaaattgtgttagattcaaaggcaaagaactaactagatcattcatccaatgtgctttctactactatattctctagttcttattgtgtcctagtagagaattctctttgctaattaatttttaacccagcatcctatattattggttctttgttcctgaagtgaatgcttgccttttttatgtttgaattgttagattgttgtggatagagaacacattgttttttggctgctttggacatgtatacctgtttttatgggtgtattgacttggatactgtttattattgcagtctttttttcaatcaagctt

SEQ ID NO: 29 - DNA, 1664 bp, synthetic construct
  misc_feature 1..1664: note = 29
  source 1..1664: mol_type = other DNA
gatccctcaacttttgattcgctatttgcagtgcacctgtggcgttcatcacatcttttgtgacactgtttgcactggtcattgctattacaaaggaccttcctgatgttgaaggagatcgaaagtaagtaactgcacgcataaccattttctttccgctctttggctcaatccatttgacagtcaaagacaatgtttaaccagctccgtttgatatattgtctttatgtgtttgttcaagcatgtttagttaatcatgcctttgattgatcttgaataggttccaaatatcaaccctggcaacaaaacttggagtgagaaacattgcattcctcggttctggacttctgctagtaaattatgtttcagccatatcactagctttctacatgcctcaggtgaattcatctatttccgtcttaactatttcggttaattaaagcacgaacaccattactgcatgtagaagcttgataaactatcgccaccaatttatttttgttgcgatattgttactttcctcagtatgcagctttgaaaagaccaaccctcttatcctttaacaatgaacaggtttttagaggtagcttgatgattcctgcacatgtgatcttggcttcaggcttaattttccaggtaaagcattatgagatactcttatatctcttacatacttttgagataatgcacaagaacttcataactatatgctttagtttctgcatttgacactgccaaattcattaatctctaatatctttgttgttgatctttggtagacatgggtactagaaaaagcaaactacaccaaggtaaaatacttttgtacaaacataaactcgttatcacggaacatcaatggagtgtatatctaacggagtgtagaaacatttgattattgcaggaagctatctcaggatattatcggtttatatggaatctcttctacgcagagtatctgttattccccttcctctagctttcaatttcatggtgaggatatgcagttttctttgtatatcattcttcttcttctttgtagcttggagtcaaaatcggttccttcatgtacatacatcaaggatatgtccttctgaatttttatatcttgcaataaaaatgcttgtaccaattgaaacaccagctttttgagttctatgatcactgacttggttctaaccaaaaaaaaaaaatgtttaatttacatatctaaaagtaggtttagggaaacctaaacagtaaaatatttgtatattattcgaatttcactcatcataaaaacttaaattgcaccataaaattttgttttactattaatgatgtaatttgtgtaacttaagataaaaataatattccgtaagttaaccggctaaaaccacgtataaaccagggaacctgttaaaccggttctttactggataaagaaatgaaagcccatgtagacagctccattagagcccaaaccctaaatttctcatctatataaaaggagtgacattagggtttttgttcgtcctcttaaagcttctcgttttctctgccgtctctctcattcgcgcgacgcaaacgatcttcaggtgatcttctttctccaaatcctctctcataactctgatttcgtacttgtgtatttgagctcacgctctgtttctctcaccacagcc

SEQ ID NO: 30 - protein, 310 aa, synthetic construct
  REGION 1..310: note = 30
MDVDVFNGWGRPRFEDESLMPPGFRFHPTDEELITYYLLKKVLDSNFSCAAISQVDLNKSEPWELPEKAKMGEKEWYFFTLRDRKYPTGLRTNRATEAGYWKATGKDREIKSSKTKSLLGMKKTLVFYKGRAPKGEKSCWVMHEYRLDGKFSYHYISSSAKDEWVLCKVCLKSGVVSRETNLISSSSSSAVTGEFSSAGSAIAPIINTFATEHVSCFSNNSAAHTDASFHTFLPAPPPSLPPRQPRHVGDGVAFGQFLDLGSSGQIDFDAAAAAFFPNLPSLPPTVLPPPPSFAMYGGGSPAVSVWPFTL

SEQ ID NO: 31 - protein, 518 aa, synthetic construct
  REGION 1..517: note = 31
MVRKRRSEWSVPEHSGSIEETGERQQQQHRGGGGGAAVSGGEDAVDDNSSSVNEGNNWRSSSRKRKDEEGEEQGDDKDEDASNLKKPRVVWSVELHQQFVAAVNQLGVEKAVPKKILELMNVPGLTRENVASHLQKYRIYLRRLGGVSQHQGNLNNSFMTGQDASFGPLSTLNGFDLQALAVTGQLPAQSLAQLQAAGLGRPAMVSKSGLPVSSIVDERSIFSFDNTKTRFGEGLGHHGQQPQQQPQMNLLHGVPTGLQQQLPMGNRMSIQQQIAAVRAGNSVQNNGMLMPLAGQQSLPRGPPPMLTSSQSSIRQPMLSNRISERSGFSGRNNIPESSRVLPTSYTNLTTQHSSSSMPYNNFQPELPVNSFPLASAPGISVPVRKATSYQEEVNSSEAGFTTPSYDMFTTRQNDWDLRNIGIAFDSHQDSESAAFSASEAYSSSSMSRHNTTVAATEHGRNHQQPPSGMVQHHQVYADGNGGSVRVKSERVATDTATMAFHEQYSNQEDLMSALLKQV

SEQ ID NO: 32 - protein, 361 aa, synthetic construct
  REGION 1..361: note = 32
MAENLACGETSESWIIDNDDDDINYGGGFTNEIDYNHQLFAKDDNFGGNGSIPMMGSSSSSLSEDRIKEMLVREIEFCPGTDYVKRLLSGDLDLSVRNQALDWILKVCAHYHFGHLCICLSMNYLDRFLTSYELPKDKDWAAQLLAVSCLSLASKMEETDVPHIVDLQVEDPKFVFEAKTIKRMELLVVTTLNWRLQALTPFSFIDYFVDKISGHVSENLIYRSSRFILNTTKAIEFLDFRPSEIAAAAAVSVSISGETECIDEEKALSSLIYVKQERVKRCLNLMRSLTGEENVRGTSLSQEQARVAVRAVPASPVGVLEATCLSYRSEERTVESCTNSSQSSPDNNNNNNNSNKRRRKQ

SEQ ID NO: 33 - protein, 630 aa, synthetic construct
  REGION 1..630: note = 33
MESDRISTPSDGTSSSLQRVRPLHGRTSGPTRRSTKGQWTTEEDEILRKAVQRFKGKNWKKIAECFKDRTDVQCLHRWQKVLNPELVKGPWSKEEDEVIVELVKKYGPKKWSTIAQHLPGRIGKQCRERWHNHLNPGINKEAWTQEEELTLIRAHQIYGNKWAELTKYLPGRTDNAIKNHWNSSVKKKLDSYLASGLLAQFPALPNVNRQNQSIPSSAKLQQSSEDDSVRKEGTEMEEASECSQGSNLAGCSQSTSDMGNKFVHTREEGKLLEDSNYRKDPSSSSAPCSEYYTPAFEDITFSMAEVPSELDESKLLEHTFSHDWAASIGKEWQFNPDDIPNISPLELMQDSSGLFMQCLTGNGNHDMVTFPQQNAVKFETTNVGSMVVGFDKPNEMFTSVEGCRMVYPEAGIPQYIPSEAGTNGADETADSLICQSSNYQISEGGNMSIENCNPLCSDVMGTSSGQPFSIPSQFSSEQSSLMFGTAANQFHNPLQGNPAQESHTSNSDGFLYPFESGTPCDNIMDDPLLEEQLDQTKDSLQLVSVNDFRTTPSNTIQTCPLVNENSSIPVEQKDGGALYYEPPRFPSLDIPFFSCDLIQSGTDAQQEYSPLGIRQLMMTSVNCLTPFRLW

SEQ ID NO: 34 - protein, 483 aa, synthetic construct
  REGION 1..483: note = 34
MSGVVRSSPGSSQPPPPPPHHPPSSPVPVTSTPVIPPIRRHLAFASTKPPFHPSDDYHRFNPSSLSNNNDRSFVHGCGVVDREEDAVVVRSPSRKRKATMDMVVAPSNNGFTSSGFTNIPSSPCQTPRKGGRVNIKSKAKGNKSTPQTPISTNAGSPITLTPSGSCRYDSSLGLLTKKFVNLIKQAKDGMLDLNKAAETLEVQKRRIYDITNVLEGIDLIEKPFKNRILWKGVDACPGDEDADVSVLQAEIENLALEEQALDNQIRQTEERLRDLSENEKNQKWLFVTEEDIKSLPGFQNQTLIAVKAPHGTTLEVPDPDEAADHPQRRYRIILRSTMGPIDVYLVSEFEGKFEDTNGSGAAPPACLPIASSSGSTGHHDIEALTVDNPETAIVSHDHPHPQPGDTSDLNYLQEQVGGMLKITPSDVENDESDYWLLSNAEISMTDIWKTDSGIDWDYGIADVSTPPPGMGEIAPTAVDSTPR

SEQ ID NO: 35 - protein, 292 aa, synthetic construct
  REGION 1..292: note = 35
MSMEMELFVTPEKQRQHPSVSVEKTPVRRKLIVDDDSEIGSEKKGQSRTSGGGLRQFSVMVCQKLEAKKITTYKEVADEIISDFATIKQNAEKPLNENEYNEKNIRRRVYDALNVFMALDIIARDKKEIRWKGLPITCKKDVEEVKMDRNKVMSSVQKKAAFLKELREKVSSLESLMSRNQEMVVKTQGPAEGFTLPFILLETNPHAVVEIEISEDMQLVHLDFNSTPFSVHDDAYILKLMQEQKQEQNRVSSSSSTHHQSQHSSAHSSSSSCIASGTSGPVCWNSGSIDTR

SEQ ID NO: 36 - protein, 241 aa, synthetic construct
  REGION 1..241: note = 36
MDSDIMNMMMHQMEKLPEFCNPNSSFFSPDHNNTYPFLFNSTHYQSDHSMTNEPGFRYGSGLLTNPSSISPNTAYSSVFLDKRNNSNNNNNGTNMAAMREMIFRIAVMQPIHIDPEAVKPPKRRNVRISKDPQSVAARHRRERISERIRILQRLVPGGTKMDTASMLDEAIHYVKFLKKQVQSLEEQAVVTGGGGGGGGRVLIGGGGMTAASGGGGGGGVVMKGCGTVGTHQMVGNAQILR

SEQ ID NO: 37 - protein, 306 aa, synthetic construct
  REGION 1..306: note = 37
MPLNGDLDRQIEQLMECKPLGEADVKILCDQAKAILVEEYNVQPVKCPVTVCGDIHGQFYDLIELFRIGGNAPDTNYLFMGDYVDAGYYSVETVSLLVALKVRYRDRLTILRGNNESRQITQVYGFYDECLRKYGNANVWKYFTDLFDYLPLTALIESQVFCLHGGLSPSLDTLDNIRSLDRIQEVPHEGPMCDLLWSDPDDRCGWGISPRGAGYTFGQDIATQFNHNNGLSLISRAHQLVMEGYNWCQEKNVVTVFSAPNYCYRCGNMAAILEIGEKMEQNFLQFDPAPRQVEPDTTRKTPDYFL

SEQ ID NO: 38 - protein, 306 aa, synthetic construct
  REGION 1..306: note = 38
MPSNGDLDRQIEQLMECKPLSEADVRTLCDQARAILVEEYNVQPVKCPVTVCGDIHGQFYDLIELFRIGGNAPDTNYLFMGDYVDAGYYSVETVSLLVALKVRYRDRLTILRGNNESRQITQVYGFYDECLRKYGNANVWKYFTDLFDYLPLTALIESQVFCLHGGLSPSLDTLDNIRSLDRIQEVPHEGPMCDLLWSDPDDRCGWGISPRGAGYTFGQDIAAQFNHNNGLSLISRAHQLVMEGFNWCQDKNVVTVFSAPNYCYRCGNMAAILEIGENMEQNFLQFDPAPRQVEPDTTRKTPDYFL

SEQ ID NO: 39 - protein, 313 aa, synthetic construct
  REGION 1..313: note = 39
MGANSIPTDATIDLDEQISQLMQCKPLSEQQVRALCEKAKEILMDESNVQPVKSPVTICGDIHGQFHDLAELFRIGGMCPDTNYLFMGDYVDAGYYSVETVTLLVALKMRYPQRITILRGNNESRQITQVYGFYDECLRKYGNANVWKIFTDLFDYFPLTALVESEIFCLHGGLSPSIETLDNIRNFDRVQEVPHEGPMCDLLWSDPDDRCGWGISPRGAGYTFGQDISEQFNHTNNLKLIARAHQLVMDGYNWAHEQKVVTIFSAPNYCYRCGNMASILEVDDCRNHTFIQFEPAPRRGEPDVTRRTPDYFL

SEQ ID NO: 40 - protein, 313 aa, synthetic construct
  REGION 1..313: note = 40
MGANSLPTDATLDLDEQISQLMQCKPLSEQQVRALCEKAKEILMDESNVQPVKSPVTICGDIHGQFHDLAELFRIGGKCPDTNYLFMGDYVDAGYYSVETVTLLVGLKVRYPQRITILRGNNESRQITQVYGFYDECLRKYGNANVWKIFTDLFDYFPLTALVESEIFCLHGGLSPSIETLDNIRNFDRVQEVPHEGPMCDLLWSDPDDRCGWGISPRGAGYTFGQDISEQFNHTNNLKLIARAHQLVMDGFNWAHEQKVVTIFSAPNYCYRCGNMASILEVDDCRNHTFIQFEPAPRRGEPDVTRRTPDYFL

SEQ ID NO: 41 - protein, 307 aa, synthetic construct
  REGION 1..307: note = 41
MPPATGDIDRQIEQLMECKALSETEVKMLCEHAKTILVEEYNVQPVKCPVTVCGDIHGQFYDLIELFRIGGSSPDTNYLFMGDYVDAGYYSVETVSLLVALKVRYRDRLTILRGNNESRQITQVYGFYDECLRKYGNANVWKHFTDLFDYLPLTALIESQVFCLHGGLSPSLDTLDNIRSLDRIQEVPHEGPMCDLLWSDPDDRCGWGISPRGAGYTFGQDIATQFNHTNGLSLISRAHQLVMEGFNWCQEKNVVTVFSAPNYCYRCGNMAAILEIGENMDQNFLQFDPAPRQVEPETTRKTPDYFL

SEQ ID NO: 42 - protein, 478 aa, synthetic construct
  REGION 1..478: note = 42
MYSGSSDGEGPDATAQRKIPPPSSMLWVRNLRRYIGSGAGLGSEALMELETKRILLDIFKEKQQKSAEAGTIPSFYKKKPEEGSISHRVQRLAKYRFLKKQSDLLLNADDLDAMWVCLRENCVIDDATGAEKMNYEDFCHIASVCTEQIGPKCRRFFSPSNFMKFEKDESGRIAILPFYLYVMRTVSLTQARIDMSELDEDSDGFLQPHEMEAYIRGLIPNLAQLRDMPAAFVQMYCRIAAHKFFFFCDPHRRGKACIKKILLSNCLQELMELHQETEEEVTDTEQAENWFSLTSAQRICDMFLALDKDMNGTLSKQELREYADGTLTDIFIERVFDEHVRRGKIGGGNAREMDFESFLDFVLALENKDAPEGLTYLFRCLDLQGRGFLTTADIHTLFRDVHQKWIEGGNYELCIEDVRDEIWDMVKPSDSLRISLADLLSCKQGGTVASMLIDVRGFWAHDNRENLLQEEEEPQEEG

SEQ ID NO: 43 - DNA, 628 bp, synthetic construct
  misc_feature 1..628: note = 43
  source 1..628: mol_type = other DNA
atctcgtctctgttatgcttaagaagttcaatgtttcgtttcatgtaaaactttggtggtttgtgttttggggccttgtataatccctgatgaataagtgttctactatgtttccgttcctgttatctctttctttctaatgacaagtcgaacttcttctttatcatcgcttcgtttttattatctgtgcttcttttgtttaatacgcctgcaaagtgactcgactctgtttagtgcagttctgcgaaacttgtaaatagtccaattgttggcctctagtaatagatgtagcgaaagtgttgagctgttgggttctaaggatggcttgaacatgttaatcttttaggttctgagtatgatgaacattcgttgttgctaagaaatgcctgtaatgtcccacaaatgtagaaaatggttcgtacctttgtccaagcattgatatgtctgatgagaggaaactgcaagatactgagcttggtttaacgaaggagaggcagtttcttccttccaaagcatttcatttgacaatgccttgatcatcttaagtagagtttctgttgtggaaagtttgaaactttgaagaaacgactctcaagtaaattgatgatcacaagtgaaagtgtatgtt

SEQ ID NO: 44 - DNA, 3963 bp, synthetic construct
  misc_feature 1..3963: note = 44
  source 1..3963: mol_type = other DNA
atgaataacggaactaataacttccaaaatttcattggtatctcttcattgcagaaaactcttagaaatgctttgattccaacagaaactacacaacagtttattgttaaaaatggtattattaaggaagatgagcttagaggtgaaaacagacaaattttgaaggatattatggatgattactacagaggttttatttctgagactttgtcttcaatcgatgatatcgattggacatcacttttcgaaaagatggagatccaattgaagaacggagataataaggatactcttattaaagaacagacagagtacagaaaggctatccataagaagtttgctaacgatgatagattcaagaacatgttctctgctaagcttatctcagatattttgcctgaattcgttatccataataacaattactctgcttcagagaaggaagagaagactcaggttattaagttgttttctagattcgctacttcttttaaggattatttcaagaacagagctaactgtttctctgctgatgatatctcttcatcttcatgtcatagaatcgttaacgataacgctgaaattttcttttctaacgctcttgtttatagaagaatcgttaagtctttgtcaaacgatgatattaataagatttctggagatatgaaggattctcttaaggaaatgtcattggaagagatctattcatacgaaaagtacggagagtttattactcaagagggtatctctttctataacgatatctgtggaaaggttaattcttttatgaatttgtactgtcaaaagaataaggagaataagaatctttataagttgcaaaagcttcataagcagattctttgtatcgctgatacatcttacgaagttccttataagtttgagtctgatgaagaggtttatcaatcagttaatggttttcttgataacatctcttcaaagcatatcgttgaaagattgagaaaaattggagataactacaatggttacaatcttgataagatctatattgtttctaagttttatgagtctgtttcacagaagacttacagagattgggaaactattaatacagctcttgagatccattacaataacattttgccaggaaatggtaaatctaaggctgataaggttaagaaagctgttaagaacgatttgcaaaagtcaatcactgaaattaatgagcttgtttctaactacaagctttgttcagatgataatattaaggctgaaacatacatccatgagatctctcatattcttaataactttgaagctcaggagttgaagtacaatcctgaaattcatcttgttgaatctgagttgaaggcttcagagcttaagaatgttttggatgttattatgaatgctttccattggtgttctgttttcatgacagaagagcttgttgataaggataataacttttatgctgaattggaagagatctatgatgagatctatccagttatttctttgtacaatcttgttagaaactacgttactcaaaagccttactcaacaaagaaaattaaacttaactttggaattccaactttggctgatggttggtctaagtcaaaggaatactctaataacgctattattcttatgagagataatttgtactaccttggaattttcaatgctaagaataagcctgataagaaaattattgaaggaaacacatcagagaataagggagattacaagaaaatgatctataatcttttgcctggtccaaataagatgatccctaaggtttttctttcttcaaagactggagttgaaacatacaaaccatctgcttacattcttgagggttacaaacaaaataagcatattaaatcttcaaaggatttcgatattactttctgtcatgatttgatcgattactttaagaactgtattgctattcatccagagtggaagaacttcggattcgatttttctgatacttcaacatacgaggatatttctggattctatagagaagttgagcttcaaggttacaagatcgattggacatacatctcagaaaaggatatcgatcttttgcaagagaaaggacagctttatttgttccagatctataataaggatttctctaagaaatcaactggtaacgataatttgcatacaatgtatttgaagaatttgttttctgaagagaatcttaaggatattgttcttaagttgaatggtgaagctgagattttctttagaaaatcttcaattaagaaccctattattcataagaaaggatctattttggttaatagaacttacgaagctgaagagaaggatcaattcggtaacatccagattgttagaaaaaatattccagaaaacatctatcaagagctttataagtacttcaatgataagtctgataaggaactttcagatgaggctgctaagttgaaaaatgttgttggacatcatgaggctgctactaatattgttaaggattacagatacacatacgacaagtattttcttcatatgcctatcactattaatttcaaggctaataagacaggtttcattaatgatagaattcttcaatacatcgctaaggaaaaggatttgcatgttatcggaatcgatagaggtgagagaaatttgatctatgtttctgttattgatacttgtggaaacatcgttgaacagaagtcattcaatatcgttaatggttacgattaccaaattaagcttaaacaacaggagggtgctagacagattgctagaaaagagtggaaggagatcggaaagattaaagaaattaaagagggttatctttctttggttattcatgaaatctcaaaaatggttattaagtacaatgctattattgctatggaggatttgtcttacggttttaagaagggtagattcaaggttgaaagacaagtttaccagaaatttgagacaatgcttattaataagttgaactatcttgttttcaaagatatctctatcactgaaaatggtggacttttgaagggataccaacttacatacatccctgataagttgaagaatgttggacatcagtgtggttgtattttctatgttcctgctgcttacacttctaaaattgatccaactacaggtttcgttaacattttcaagtttaaagatttgacagttgatgctaagagagagtttattaagaagttcgattctatcagatacgattcagagaaaaatcttttctgtttcactttcgattacaataactttattactcaaaatacagttatgtctaagtcttcatggtcagtttacacatatggagttagaattaaaagaagatttgttaatggtagattctctaatgagtcagatactatcgatatcacaaaggatatggaaaagactttggagatgacagatattaattggagagatggtcatgatcttagacaagatatcatcgattacgaaattgttcagcatatcttcgagattttcagacttactgttcagatgagaaattctttgtcagaacttgaggatagagattacgatagacttatctctcctgttttgaatgagaataacattttctatgattcagctaaggctggagatgctttgccaaaagatgctgatgctaatggtgcttactgtattgctttgaagggtctttacgagattaaacaaatcacagaaaactggaaagaggatggaaagttttctagagataagcttaagatctcaaataaggattggttcgatttcattcagaataagagatacttgaaaaggccagcagcaaccaaaaaggcaggacaggcaaagaagaagaaaggatcttatccttatgatgttcctgattatgctggatatccttatgatgttcctgattatgctggatcttatccttatgatgttcctgattatgctggatctcctaaaaagaaaagaaaggtttaa

SEQ ID NO: 45 - DNA, 864 bp, synthetic construct
  misc_feature 1..864: note = 45
  source 1..864: mol_type = other DNA
ccgatccattcggtccccagattagccttttcaatttcagaaagaatgctaacccacagatggttagagaggcttacgcagcacgtctcatcaagacgatctacccgagcaataatctccaggaaatcaaataccttcccaagaaggttaaagatgcagtcaaaagattcaggactaactgcatcaagaacacagagaaagatatatttctcaagatcagaagtactattccagtatggacgattcaaggcttgcttcacaaaccaaggcaagtaatagagattggagtctctaaaaaggtagttcccactgaatcaaaggccatggagtcaaagattcaaatagaggacctaacagaactcgccgtaaagactggcgaacagttcatacagagtctcttacgactcaatgacaagaagaaaatcttcgtcaacatggtggagcacgacacacttgtctactccaaaaatatcaaagatacagtctcagaagaccaaagggcaattgagacttttcaacaaagggtaatatccggaaacctcctcggattccattgcccagctatctgtcactttattgtgaagatagtggaaaaggaaggtggctcctacaaatgccatcattgcgataaaggaaaggccatcgttgaagatgcctctgccgacagtggtcccaaagatggacccccacccacgaggagcatcgtggaaaaagaagacgttccaaccacgtcttcaaagcaagtggattgatgtgatatctccactgacgtaagggatgacgcacaatcccactatccttcgcaagacccttcctctatataaggaagttcatttcatttggagagaacacgggggacgagct

SEQ ID NO: 46 - DNA, 43 bp, synthetic construct
  misc_feature 1..43: note = 46
  source 1..43: mol_type = other DNA
aaattactgatgagtccgtgaggacgaaacgagtaagctcgtc

SEQ ID NO: 47 - DNA, 20 bp, synthetic construct
  misc_feature 1..20: note = 47
  source 1..20: mol_type = other DNA
taatttctactgttgtagat

SEQ ID NO: 48 - DNA, 20 bp, synthetic construct
  misc_feature 1..20: note = 48
  source 1..20: mol_type = other DNA
tatgtaggtgtatttggaat

SEQ ID NO: 49 - DNA, 68 bp, synthetic construct
  misc_feature 1..68: note = 49
  source 1..68: mol_type = other DNA
ggccggcatggtcccagcctcctcgctggcgccggctgggcaacatgcttcggcatggcgaatgggac

SEQ ID NO: 50 - DNA, 299 bp, synthetic construct
  misc_feature 1..299: note = 50
  source 1..299: mol_type = other DNA
agcggccgcccggctgcagatcgttcaaacatttggcaataaagtttcttaagattgaatcctgttgccggtcttgcgatgattatcatataatttctgttgaattacgttaagcatgtaataattaacatgtaatgcatgacgttatttatgagatgggtttttatgattagagtcccgcaattatacatttaatacgcgatagaaaacaaaatatagcgcgcaaactaggataaattatcgcgcgcggtgtcatctatgttactagatccgatgataagctgtcaaacatgagaatt

SEQ ID NO: 51 - DNA, 933 bp, synthetic construct
  misc_feature 1..933: note = 51
  source 1..933: mol_type = other DNA
atggatgttgatgtattcaatggatggggtagacctagatttgaagatgaatctttgatgcctccaggattcaggtttcaccctactgatgaagaactaataacatattatcttctgaagaaggtcttagactcgaatttttcatgtgcagctatctcacaggtggatttgaacaaatcagagccatgggaactccctgaaaaagcaaagatgggagagaaagagtggtatttcttcaccctccgtgacagaaaatatccgacagggctacggacaaacagagccactgaagctggttattggaaagctactggaaaagatcgagagataaaatcttctaagaccaaatcactgcttggcatgaagaaaacacttgttttctacaagggccgcgcaccaaaaggggagaagagttgttgggtgatgcatgaatataggttggatggaaagttttcttaccactacatttcatcatctgccaaggatgagtgggttctttgcaaagtttgtcttaaaagtggtgtggtaagtagagagacaaatttgatttcctcctccagctcttctgcagttactggtgaatttagctcagccgggtccgcaattgctccaataatcaatacctttgctacggaacatgtatcttgcttcagcaacaattctgcagctcatactgacgcatcatttcatacatttttaccagctcctcccccgagtttgcctccacgtcaaccaaggcatgtgggtgatggtgttgcttttggtcaatttcttgacctcggctcgtcgggccagattgattttgatgctgcggccgcagcatttttccctaatttaccctcattgcccccaactgtcctgccaccacctcctagttttgctatgtatggtggaggaagtcccgctgtctctgtttggcctttcactttatga

SEQ ID NO: 52 - DNA, 1557 bp, synthetic construct
  misc_feature 1..1557: note = 52
  source 1..1557: mol_type = other DNA
atggtaagaaagagaaggagtgagtggagcgttccagagcactcaggttcaatcgaagaaactggagagcggcagcagcagcagcatcgtggaggaggtggtggtgctgctgtgtcgggaggtgaagatgcggttgatgataattccagtagtgtaaatgagggcaacaattggagatcgtcctcaaggaaaaggaaggatgaagaaggtgaggagcaaggtgatgataaagatgaggatgcatctaatttgaaaaagcctagagttgtttggtctgttgaattgcatcagcaatttgttgctgcagtaaaccaactcggcgtcgagaaagcagtcccaaagaagatccttgaattaatgaatgttcctggattaaccagagaaaatgtggcctctcaccttcagaaatatcgtatctacttaaggaggctgggtggcgtgtctcaacaccaagggaacttaaacaacagtttcatgactggtcaagatgcttcatttggtcctctttctacacttaatgggtttgacttgcaggcacttgccgttacaggacaactgcctgctcagtctttagctcaactacaagcagcagggttgggccggcctgcaatggtgtctaaatctggattgcctgtgtcgtcaattgttgacgaaagatcaatattctcttttgataacacaaagacaagatttggagaaggacttggccatcatggtcagcaaccacaacaacaaccacaaatgaacctcctccatggagtacctactggactgcaacagcagctacctatgggaaacagaatgtcaattcaacagcaaattgctgcggtacgagctggaaattcagtgcaaaacaatggaatgctgatgccattggcagggcagcaatcactgccaagaggtcccccgccaatgcttactagctcgcagagctccataaggcagcccatgttgtccaatcgtatttctgagcgcagcgggttcagtggaaggaataatataccagaatcatcgcgagttctccctacgagttatacaaatcttacgacacagcactcatcatctagtatgccttacaacaatttccagcctgagttgccggtgaattctttccccttggcctctgctccgggtatatctgtgcctgttcgtaaagctactagttaccaagaggaagtcaattccagcgaggctggttttaccactccatcctatgatatgtttacaactagacagaatgattgggatcttagaaacattggaattgcattcgacagtcatcaagacagtgaatctgcagcattttcagcgtcagaagcttattcttccagctcaatgagtagacataatactactgttgccgcaactgaacatgggcgaaatcatcaacagccaccatcaggcatggttcaacatcaccaggtttatgctgatggaaatggtgggtcagttcgcgtcaaatccgagagggtagccaccgatacagcaacaatggcttttcatgaacaatatagtaatcaagaagatcttatgtcagctttattgaagcaagtctga

SEQ ID NO: 53 - DNA, 1086 bp, synthetic construct
  misc_feature 1..1086: note = 53
  source 1..1086: mol_type = other DNA
atggctgaaaatcttgcttgtggtgagacttctgaatcatggattattgataatgatgatgatgacattaactatggaggaggcttcacaaatgaaatagattacaatcatcaactttttgcaaaagacgacaattttggtggaaacgggtcaataccaatgatgggatcttcatcttcatcgctaagtgaagatagaataaaggaaatgttggtgcgtgaaattgagttttgtccaggaacagattatgtcaaaaggctattgtcaggagatttagacctttcggtaagaaatcaagctcttgactggatattgaaagtttgtgctcattatcattttgggcacctttgcatttgtctgagtatgaattatttggaccgcttcctgacctcttatgaattaccgaaggataaagattgggctgcacagctcttggcagtgtcgtgcctaagcctagcatctaaaatggaagaaactgatgttcctcacattgtggatctccaagttgaggatccaaaatttgtatttgaggccaagacaatcaagagaatggagcttctggttgttaccactttgaattggagattacaggcacttactccattctctttcattgactactttgttgataagatttctggccatgtctccgagaacttgatataccggagttcccgatttatccttaatacaacaaaagctattgaatttctcgatttcaggcccagcgagattgctgcggctgcggctgtcagtgttagtatctctggtgaaacagaatgtatcgatgaagagaaggcattgtcatccctgatatatgtaaagcaagagagagtgaaaagatgtttaaatttgatgagatctttaactggggaagaaaatgttaggggtacaagtctatctcaagaacaagcaagggttgctgttcgtgccgtacctgccagccctgttggtgtactggaggcaacttgccttagctaccgttcagaggaaagaacggtggagtcatgcactaattctagccagagttcacctgataacaacaataataataacaattcaaacaaaaggcgccgaaagcagtga

SEQ ID NO: 54 - DNA, 1893 bp, synthetic construct
  misc_feature 1..1893: note = 54
  source 1..1893: mol_type = other DNA
atggaaagtgatcgtatctcaaccccctccgatggcacatcttcctccctacaaagagttaggccacttcatggacgtacgagcggacccacacgacggtccactaaaggtcaatggacaactgaagaggatgagatactgagaaaggcagttcaacggttcaaggggaagaattggaaaaaaatagctgaatgttttaaagatagaaccgacgtgcagtgtttgcataggtggcaaaaggtgctgaacccagagcttgtgaagggcccatggtcaaaagaggaagatgaagttattgttgagctggttaagaagtatgggcctaagaaatggagtacaattgcacaacatcttccaggaaggataggcaaacaatgccgcgaaagatggcataaccatttgaatcctggtatcaacaaagaagcctggactcaggaggaagaacttactttaataagggctcatcagatttatggaaataagtgggcagagttgactaaatatttgccgggacgaactgataatgcaattaaaaatcattggaattcatctgttaagaaaaagcttgatagttacttagcgagcgggctcctagcccaatttcctgctttaccaaatgtaaacaggcaaaatcaaagcattccgagttcagcaaaactgcagcagtcatccgaagatgattccgtaaggaaggagggcacagaaatggaggaagcatctgaatgttcacaaggttctaatttggcgggatgttctcaaagtacgtcagacatgggaaacaagtttgtacataccagagaggagggtaaacttctcgaggactcgaattatagaaaagacccatcaagctcttcggctccttgcagcgaatattatacacctgcatttgaagatatcaccttttccatggctgaggttcctagtgaattagatgaatcaaagttactagaacatactttctcacatgattgggctgctagtattggtaaggaatggcagttcaatcctgatgacattcccaacatttctccacttgagttaatgcaagattcttctggtttgttcatgcagtgcttgactggcaatggtaatcacgatatggtaacatttccacagcaaaacgctgtcaaatttgagacaacaaatgttggatcaatggtggtgggatttgataaacctaatgagatgttcacatcagttgaaggttgtagaatggtttaccctgaagctgggataccacaatacatcccatctgaggctggaactaatggggcagatgaaactgctgattcactgatttgtcaatcgagtaactatcaaatctcagaaggaggtaatatgtcaattgaaaattgcaacccactctgctctgatgtcatgggtacttcttctggccaacctttctcaatcccttctcagttttcctccgagcagtctagtttgatgtttggtactgcagcaaatcagtttcacaatcccctgcaaggaaacccagctcaggagtctcacacaagtaactcagatggttttttgtatccatttgaaagtggaactccatgtgataacataatggatgatcctctactcgaagagcagttggatcaaacaaaggattctcttcagctcgtttctgtcaatgattttcgtacgaccccttccaatacaattcagacttgtccattggtaaatgaaaactcgtctataccggtggaacaaaaagacggaggtgccctttactatgaaccaccccgcttcccttctctagacatccctttcttctcatgtgaccttattcaaagtgggacagatgctcaacaagaatactctcctttgggtattagacagctcatgatgacttcagttaattgcttaactccgtttagattgtggtga

SEQ ID NO: 55 - DNA, 1452 bp, synthetic construct
  misc_feature 1..1452: note = 55
  source 1..1452: mol_type = other DNA
atgagcggggtcgtacgttcgtcccctggaagtagtcagcctcccccccctccgcctcaccaccctcctagttccccagtccctgtaacgtccactccagttattccaccaatacgccgacatttggcatttgcttctactaaacctccatttcatccatcagatgattatcataggttcaatccttctagtttgtctaataacaatgatagaagtttcgttcatggttgtggtgttgttgatcgggaagaagatgcagtggtagtgagatctccttcgagaaaaagaaaggccacaatggatatggtggtggctccatcaaataatgggtttacttcttcaggcttcacaaacataccgtctagtccttgtcagacaccacgtaaaggtggaagggttaatattaagtcaaaggccaagggaaacaaaagcacgccacagacccctatctccaccaatgctggatcgccaatcactttaaccccgtctgggtcatgcaggtacgattctagccttggactgctcacgaagaaatttgtgaatttgattaaacaagcaaaggatggaatgttagatttgaacaaagcagctgaaactcttgaggttcaaaagaggcgtatatatgacattacaaatgtgcttgaaggtattgatctcattgaaaagccattcaagaacagaatcttatggaagggggtggatgcttgtcctggagatgaggatgccgacgtatcagtcctccaagcagagatcgaaaacttagctcttgaggagcaggcgttggataatcaaattcggcaaactgaagagagactaagagatctatcagagaatgaaaaaaaccagaaatggctttttgttactgaggaagatataaaaagtctgccaggatttcaaaatcagacattgattgcagttaaagcaccgcacggtactactctggaggttccagatcctgatgaagcagcagatcatccacaaaggagatatagaataattcttcgctcgactatgggccctattgatgtttacctggtatctgaatttgaaggaaagtttgaggacacaaatggttctggtgctgcgcccccagcttgccttcctattgcatctagctctggctcaacaggtcatcatgatatcgaagctctaacagtggacaaccctgaaacagctattgtatcacatgatcaccctcatccccaaccaggtgatactagtgacctcaattatttgcaggagcaagttggaggtatgttaaagatcacaccaagtgatgttgaaaatgacgaatctgactattggctactttccaatgcagagatatcaatgacagacatatggaaaactgattcaggcatagattgggattacggaatcgctgatgtcagcacaccacctcctgggatgggagaaattgcccctactgctgttgactcaaccccacgatga

SEQ ID NO: 56 - DNA, 879 bp, synthetic construct
  misc_feature 1..879: note = 56
  source 1..879: mol_type = other DNA
atgagcatggaaatggagttatttgtgacacctgaaaaacagcgtcagcatccatcagtaagtgtagaaaaaactccggtacgaaggaaattgattgttgatgacgacagtgaaattgggtctgaaaagaaaggacagagtcggacttcaggtggtggattgaggcaattttcagtgatggtgtgtcagaagctagaggcgaaaaaaataaccacatataaagaggttgctgatgaaataatctctgattttgcaacaatcaaacaaaatgctgagaaaccattaaacgaaaatgagtataatgagaagaacattaggagaagagtttatgatgcactgaatgtttttatggctttggatataatcgccagagacaaaaaagaaatcaggtggaaagggctcccaattacttgtaagaaggatgttgaagaagttaaaatggacagaaacaaggttatgagtagcgttcagaaaaaggcagcatttcttaaggaacttcgcgagaaagttagttcgcttgaatcattgatgtcaagaaatcaagagatggtagttaaaactcaaggtcctgctgaaggatttactttaccctttatactactggaaacaaatcctcatgctgttgttgagattgagatatcagaagatatgcaactcgtccaccttgatttcaatagcacgcctttctctgttcatgatgatgcttacattttgaagctaatgcaggaacaaaagcaagaacagaaccgtgtctcttcctcatcgtccactcatcatcaatctcaacattcttctgcccactccagttcaagttcttgcattgcatctggaacttctggcccagtatgttggaattctggttcaattgatactcgatga

SEQ ID NO: 57 - DNA, 726 bp, synthetic construct
  misc_feature 1..726: note = 57
  source 1..726: mol_type = other DNA
atggattctgatattatgaatatgatgatgcatcagatggagaagcttccagagttctgcaatccgaactcttcatttttttctcctgatcataataacacatatccatttctcttcaattcaactcattaccagtcagaccacagcatgacaaatgaacctggatttcgttatggtagcggcttgttaaccaatccctcctccataagcccaaatacagcctacagttcggtttttcttgataaaagaaataattccaacaacaacaataatggaacgaacatggctgctatgagagaaatgattttcagaattgcagtgatgcaacctattcacatagatccagaagcagtaaaacctccaaagagaaggaatgttaggatctcaaaagatcctcagagtgtagcagccagacatcggagagagaggatatctgaaaggatccggatcttgcagcgtctagtaccggggggtactaaaatggacactgcttcaatgttggatgaagctattcattatgttaaatttctgaagaagcaagttcaatctctggaggaacaagctgtcgtcactggtggtggaggaggtggtggggggcgtgtgttaataggagggggtggaatgactgcagcgagtggtggcggcggaggcggtggtgttgttatgaaggggtgtggaaccgtgggaacacatcaaatggttggaaatgctcaaattcttcgatga

SEQ ID NO: 58 - DNA, 921 bp, synthetic construct
  misc_feature 1..921: note = 58
  source 1..921: mol_type = other DNA
atgcccttgaatggagatcttgatagacagattgaacaattgatggaatgcaaaccacttggagaagctgatgtgaagattttgtgtgatcaagcaaaagcaatcctggtagaagagtacaatgttcagcctgtaaagtgtccagtgaccgtgtgtggtgacattcatgggcagttttacgacctgatcgagcttttcaggatcggaggaaatgctcctgacaccaactatctcttcatgggtgattatgttgatgccggctattacagcgtagaaactgttagtcttttagttgctcttaaagtaagatacagagatcggctaacaattctacgcggaaacaacgaaagtagacaaatcactcaagtctatggattttatgatgagtgtcttagaaaatatgggaatgcaaacgtttggaagtatttcactgatttgtttgactatcttccgctcacggccctaatagagtcacaggttttttgcctccacggtggcttgtctccttcactagatactttggacaatatccggtccttggatcgtattcaagaagttccccatgaaggtcctatgtgtgacttactttggtctgatccagatgatcgatgtggatggggaatatcgccaagaggagctggttatacgtttggtcaagatatagcgacacaattcaaccacaacaatggtttatcattaatatctagagctcatcaactcgtgatggaaggctacaactggtgccaagagaaaaatgtcgtcaccgttttctccgctccgaattactgttaccgttgcgggaacatggcagctattctggagattggcgagaagatggagcagaattttctccagtttgatcctgcgccgaggcaggtggagccagacacaactagaaagactcctgattacttcctgtga

SEQ ID NO: 59 - DNA, 921 bp, synthetic construct
  misc_feature 1..921: note = 59
  source 1..921: mol_type = other DNA
atgccttccaatggagatcttgaccggcagattgagcagctgatggaatgcaagcccttaagtgaagctgatgtaaggacgctttgtgatcaggccagagctatcttggtcgaagaatacaatgttcagcctgtcaaatgtcctgttacagtttgcggtgatattcatggacagttttacgacttgattgaattatttcgtatcggaggtaacgccccagacacaaattatttattcatgggtgattatgtagatgcgggatactattccgtggaaactgttagccttctcgtcgcgctaaaggttagatacagggataggttgacaatcttgagaggaaacaacgaatctcgccagataacccaagtgtatggattctatgatgagtgccttaggaagtatggcaatgctaatgtgtggaaatattttactgatctcttcgattacctcccgttaacagctctcattgagtcgcaagttttttgcctacacggtgggctctcacctagccttgacactttggataacattcgttctctggatagaatacaagaagttccacatgaggggccaatgtgtgatcttttgtggtctgaccctgatgatagatgtggttgggggatcagtccgcgaggtgcaggatatacattcgggcaagatatcgccgcacaattcaatcacaacaatggtctgtcactcatatctcgagctcatcaactcgttatggagggattcaattggtgtcaagacaagaacgtggtgaccgtcttttcagctccaaactattgttaccggtgtggaaacatggcagcaatacttgagattggcgaaaatatggagcaaaattttctacagtttgatcccgctccaagacaagtagagccagatactactagaaaaacgcctgactactttctttga

SEQ ID NO: 60 - DNA, 942 bp, synthetic construct
  misc_feature 1..942: note = 60
  source 1..942: mol_type = other DNA
atgggagcaaattccattccaaccgacgctacgattgatctagatgaacaaatcagtcagctcatgcaatgcaaaccattaagtgaacagcaagtgagagccctttgtgagaaagcaaaagagatattgatggacgagtcaaatgttcagcctgttaagtcgccggtaaccatatgtggagacattcatggacaatttcatgatcttgcagagctcttcaggatcggaggtatgtgccccgacacaaattacttgttcatgggtgattatgtggatgcaggctattactctgtggaaactgtaactctccttgtcgcgctcaagatgagataccctcagaggataaccattctgcgcggaaacaacgaatcaagacagataacacaagtttatggtttttatgatgagtgcttacgtaagtatggcaatgctaatgtctggaagatcttcactgatctgtttgattactttcctctaactgctcttgttgaatctgaaatcttttgtttgcacggcgggctcagtccctcaatagaaacacttgataacatccggaattttgaccgtgtccaagaagtacctcatgaaggtccaatgtgtgatttattgtggtctgatcctgatgacaggtgtggttggggaatcagcccgcgaggagccgggtacacatttggtcaagatatttccgagcaattcaaccatacaaacaatttgaaactaattgcaagagctcatcaattggtgatggatggttacaattgggctcacgagcagaaagttgtgacaattttctctgctccaaactattgctatagatgtgggaatatggctagcatccttgaggttgatgattgtcgtaaccacactttcattcagtttgagccagcgcctcgaagaggagaaccagatgttactcggagaacgccggactatttcttgtga

SEQ ID NO: 61 - DNA, 942 bp, synthetic construct
  misc_feature 1..942: note = 61
  source 1..942: mol_type = other DNA
atgggagctaattcgctgccgacagatgcaacattggacttggatgagcaaatctctcagctaatgcaatgcaaaccattatcagaacaacaagtcagagccctctgtgagaaggctaaagaaattctcatggatgagtcaaatgtgcagcctgtcaaatccccggttacaatatgtggcgatattcatggtcaatttcatgatcttgctgagttattcagaatcggtggtaaatgccctgataccaactacctcttcatgggtgattatgtggatgctggttactacagcgttgaaactgtgactctactagtaggcctcaaagttagatatcctcaaagaattaccattctgcggggaaacaatgaaagcaggcagattactcaagtatatggtttctatgatgaatgtctgaggaagtatggaaatgcaaatgtttggaagattttcactgacctatttgactactttcctcttacagcgttggtcgagagtgagatattttgtttgcatggggggctctcaccttccattgaaacccttgacaatatcagaaactttgatagagttcaagaagttcctcatgaaggaccaatgtgtgatttgctttggtctgatccagacgaccgttgcggatggggaatcagtccccgtggcgccggatacacatttgggcaagatatatctgaacagttcaatcacacaaacaacttgaagcttatagcaagggcccatcagcttgtgatggacgggtttaactgggctcatgagcagaaggttgtaacgatcttctcagcgccaaattactgttatagatgtggtaacatggcttctatcttggaggttgatgattgccgtaaccacactttcattcagtttgagccagcaccccgacgaggagaaccagatgtgacgaggcgcactcctgactatttcttatga

SEQ ID NO: 62 - DNA, 924 bp, synthetic construct
  misc_feature 1..924: note = 62
  source 1..924: mol_type = other DNA
atgccaccggccactggtgatatagataggcagatcgaacaattgatggagtgcaaagcgctgagcgagactgaggtaaagatgctttgtgaacacgccaaaaccattctcgttgaagaatacaatgttcaacctgtgaaatgtcccgtcaccgtttgtggggacattcacggtcagttttatgatctgattgaactctttagaattgggggctcatctcctgatactaactatttattcatgggagattatgttgatgctggttactatagcgtggagacagtatctctattggttgcattgaaagtcagataccgtgaccgtctaacaatattacgggggaataatgagtcacgacagattacacaggtctatggcttctacgacgaatgtcttagaaagtatggaaatgctaacgtttggaaacatttcactgatctttttgattaccttcctctcactgcactgattgagtctcaggttttctgcttacatggaggtcttagtccctcactagacacgcttgataacatccgctccctcgaccgaatccaagaagttcctcatgaaggtccaatgtgtgatttgttgtggtctgatccagatgatagatgtggttggggaatctcgccaagaggagctggatatacctttggacaagatatagcaactcaatttaaccacacaaatggtttatccttaatcagtagagctcatcagcttgtgatggaggggttcaattggtgtcaagagaagaatgtagtcacggtgtttagtgctccaaactactgctacagatgcggaaacatggctgcaatacttgagattggtgagaatatggatcaaaacttcttgcagttcgatcctgcgccgaggcaagtggaacctgaaacaacgagaaagactccagactattttctctga

SEQ ID NO: 63 - DNA, 1437 bp, synthetic construct
  misc_feature 1..1437: note = 63
  source 1..1437: mol_type = other DNA
atgtacagtggctcaagcgatggagaaggtcctgacgctacggcgcaacgaaagattcccccgccatcctcaatgctttgggttcgaaacctccgaagatacatcggatccggtgcgggtctcgggtctgaagccctaatggagcttgaaacaaaaagaatattgctagatatttttaaggagaagcaacaaaagagtgctgaagctggcacaattcctagcttttataagaagaaacctgaagagggatctatcagtcatagggttcagaggttggcaaaataccgatttttaaagaaacaatctgaccttttgctgaatgctgatgatttggatgctatgtgggtatgcctaagagaaaactgtgtgatagatgatgcaactggtgcagaaaagatgaattatgaagacttttgccacattgcctctgtatgtacagaacaaatagggcctaaatgtcgccgctttttcagtccttcaaatttcatgaagtttgagaaggatgaatcagggaggattgccatcctgccattttacctatatgtgatgcgtacagtttcacttactcaagcccgaattgacatgagtgagcttgatgaagactctgatggtttccttcaaccccatgaaatggaagcctatatacggggcctgattcctaacctagcacagcttcgagacatgccagcagcttttgtccaaatgtattgccgtatagctgcacacaaatttttcttcttttgtgatccccataggcgaggtaaggcatgcataaaaaagattttacttagcaactgtctccaagagttgatggaacttcaccaggaaactgaggaggaagttactgacacagagcaagctgaaaactggttttccttgacttctgcacagaggatttgtgacatgtttcttgctcttgataaagatatgaatggaacattgagcaagcaggagctaagggaatatgcggatggtacactaacagatatcttcattgaaagagtttttgatgagcatgttcgacgtggaaaaattggaggcggcaatgcccgtgaaatggattttgaaagtttccttgacttcgttctagccctggaaaacaaggatgccccggagggtcttacatatttgttcaggtgtcttgatctccaaggaaggggtttcttaactacagcggatattcacacactattcagagatgtccatcaaaaatggattgaaggagggaactatgaactatgcatcgaggatgtaagggatgaaatatgggatatggtgaagccgtctgactctttgaggatatcactggctgatttgctatcatgcaaacaaggtggcactgttgcaagcatgcttatagatgtgcgtggtttctgggcccatgacaacagagaaaatcttctacaggaagaggaagaaccccaagaagaaggatga

SEQ ID NO: 64 - DNA, 400 bp, synthetic construct
  misc_feature 1..400: note = 64
  source 1..400: mol_type = other DNA
gactctgatggtttccttcaaccccatgaaatggaagcctatatacggggcctgattcctaacctagcacagcttcgagacatgccagcagcttttgtccaaatgtattgccgtatagctgcacacaaatttttcttcttttgtgatccccataggcgaggtaaggcatgcataaaaaagattttacttagcaactgtctccaagagttgatggaacttcaccaggaaactgaggaggaagttactgacacagagcaagctgaaaactggttttccttgacttctgcacagaggatttgtgacatgtttcttgctcttgataaagatatgaatggaacattgagcaagcaggagctaagggaatatgcggatggtacactaacagatatcttcattgaaa

SEQ ID NO: 65 - DNA, 1627 bp, synthetic construct
  misc_feature 1..1627: note = 65
  source 1..1627: mol_type = other DNA
gcccttggtaaggaaataattattttcttttttccttttagtataaaatagttaagtgatgttaattagtatgattataataatatagttgttataattgtgaaaaaataatttataaatatattgtttacataaacaacatagtaatgtaaaaaaatatgacaagtgatgtgtaagacgaagaagataaaagttgagagtaagtatattatttttaatgaatttgatcgaacatgtaagatgatatacggccggtaagaggttccaactttcaccataatgaaataagatcactaccgggcgtattttttgagttatcgagattttcaggagctaaggaagctaaaatggagaaaaaaatcactggatataccaccgttgatatatcccaatggcatcgtaaagaacattttgaggcatttcagtcagttgctcaatgtacctataaccagaccgttcagctggatattacggcctttttaaagaccgtaaagaaaaataagcacaagttttatccggcctttattcacattcttgcccgcctgatgaatgctcatccggaattccgtatggcaatgaaagacggtgagctggtgatatgggatagtgttcacccttgttacaccgttttccatgagcaaactgaaacgttttcatcgctctggagtgaataccacgacgatttccggcagtttctacacatatattcgcaagatgtggcgtgttacggtgaaaacctggcctatttccctaaagggtttattgagaatatgtttttcgtctcagccaatccctgggtgagtttcaccagttttgatttaaacgtggccaatatggacaacttcttcgcccccgttttcaccatgggcaaatattatacgcaaggcgacaaggtgctgatgccgctggcgattcaggttcatcatgccgtctgtgatggcttccatgtcggcagaatgcttaatgaattacaacagtactgcgatgagtggcagggcggggcgtaatcgcgtggatccggcttactaaaagccagataacagtatgcgtatttgcgcgctgatttttgcggtataagaatatatactgatatgtcggtcccataatagtaattctagctggtttgatgaattaaatatcaatgataaaatactatagtaaaaataagaataaataaattaaaataatatttttttatgattaatagtttattatataattaaatatctataccattactaaatattttagtttaaaagttaataaatattttgttagaaattccaatctgcttgtaatttatcaataaacaaaatattaaataacaagctaaagtaacaaataatatcaaactaatagaaacagtaatctaatgtaacaaaacataatctaatgctaatataacaaagcgcaagatctatcattttatatagtattattttcaatcaacattcttattaatttctaaataatacttgtagttttattaacttctaaatggattgactattaattaaatgaattagtcgaacatgaataaacaaggtaacatgatagatcatgtcattgtgttatcattgatcttacatttggattgattacagttggtctagagatttcgtctaga

SEQ ID NO: 66 - DNA, 94 bp, synthetic construct
  misc_feature 1..94: note = 66
  source 1..94: mol_type = other DNA
gtctatttaactcagtattcagaaacaacaaaagttcttctctacataaaattttcctattttagtgatcagtgaaggaaatcaagaaaaataa

SEQ ID NO: 67 - DNA, 3858 bp, synthetic construct
  misc_feature 1..3858: note = 67
  source 1..3858: mol_type = other DNA
atgtctaaattggagaagttcacaaattgttactcactctctaaaactttgaggtttaaagctataccagtgggaaaaacgcaagaaaatattgataacaagagactcctggtagaagatgaaaaaagggctgaagattacaaaggtgtaaagaagttgctagatagatactatttgtcattcattaatgatgttcttcacagcatcaaactgaaaaatttgaacaattatattagtctcttcagaaagaaaacaaggactgagaaagaaaacaaagagctagagaacctcgaaataaatttaagaaaagaaattgccaaagcattcaagggaaatgaaggatacaaaagtctttttaagaaggacataattgaaaccatcttacccgagtttcttgatgacaaggatgaaatagcactcgtcaattctttcaatggtttcaccactgcatttactggttttttcgataatagagagaacatgttttccgaggaagcaaaaagtacaagcatcgcttttcgctgcattaatgagaatttgactagatatatatccaatatggatatcttcgagaaggttgatgcgatttttgacaaacatgaagtgcaggagattaaagagaaaatattgaattctgattatgatgtagaagacttctttgagggcgagttcttcaattttgtgcttactcaagaaggtattgatgtatacaatgcaattatagggggctttgttactgagtctggtgaaaagataaagggattgaatgagtatatcaacttgtataatcagaagacaaaacagaaacttccaaagtttaaaccactttataagcaggttctaagtgatcgtgagtccctgagtttctatggggagggatatactagtgacgaagaagttttggaagtttttcgtaataccttgaataaaaactccgaaattttctcttcaataaagaaacttgagaagttattcaaaaactttgatgagtattcttctgcaggcatctttgttaaaaatggacctgcaatatcgactataagcaaagatatttttggcgaatggaatgtcattagggataagtggaacgcagaatacgatgatattcatttgaaaaaaaaagctgtagttacggaaaagtatgaggatgataggaggaaaagctttaagaaaattggttccttttctctggaacaactacaggaatatgccgatgccgacctcagtgttgttgaaaaattaaaggaaatcatcattcagaaggttgatgagatctataaagtctatggttcatctgaaaaactatttgatgcagatttcgtgttagagaaaagcctgaagaagaacgacgctgttgttgctatcatgaaggatttgctggactccgtgaagtcattcgaaaattacatcaaagccttctttggagaaggcaaagagactaatcgagatgaaagtttttatggagattttgtccttgcttacgacattctcttgaaagttgatcacatttatgatgcgatccgtaactatgttacacagaagccctactctaaagataagtttaagttatatttccaaaaccctcagtttatgggtggttgggataaagataaagaaacggactatagagctactatcttgcgttatggttccaagtattatttagcaatcatggataaaaagtacgccaagtgccttcaaaagatagataaagacgatgtaaatgggaactatgaaaaaatcaactataaactgctgccgggaccaaataaaatgcttcctaaagtctttttctcaaaaaagtggatggcttactacaacccaagtgaagatattcagaaaatatataagaatggaacattcaaaaagggggatatgttcaatcttaatgattgtcataagttgattgatttttttaaggatagtatatctcgatatcccaaatggagtaatgcatatgattttaatttctcagaaacagaaaaatacaaggatattgccggattctacagagaagttgaggagcagggttacaaggtatcttttgaatcagcaagtaagaaagaagtggataaactagtggaagaagggaagctttatatgtttcaaatctacaacaaagatttttcggataagtctcacggaactcctaatcttcatacaatgtactttaaattactgtttgatgagaacaaccatggtcaaattagactatctggaggagctgaactttttatgagaagagcttctctcaaaaaagaggagcttgttgttcatccagcaaattccccaatcgcaaataagaatcctgacaatccaaaaaaaaccactacattaagttatgacgtttacaaagataaacgattttcagaagatcaatacgaattgcatattcctattgctatcaacaaatgtcctaagaatatattcaagataaatactgaagttcgtgttctgctgaaacacgatgataatccgtatgttattggcattgaccgcggtgaaaggaatcttctctatattgtggtggtcgatgggaaagggaacattgtggaacaatattccttaaatgaaatcattaataatttcaacggtataaggatcaagaccgactatcattcgttgcttgacaagaaagagaaggagagattcgaggctcgccagaattggactagcattgagaatataaaagaattaaaagctggctacatatcacaagtcgtgcacaagatctgtgaacttgtagagaagtatgatgctgtgattgctctagaggacctcaatagtggtttcaagaactctagagtgaaagtggaaaagcaagtttatcaaaaatttgagaagatgctgattgataaactaaactacatggttgacaaaaaatctaacccttgtgcgactggaggggctctgaagggttatcagattaccaataaattcgagtcatttaagagcatgtcaactcaaaatggcttcatattttacattcctgcatggttgacatcaaagatagacccatctacaggatttgtaaatttactaaagaccaagtacacatctatcgccgacagtaagaagtttatatcatcttttgataggattatgtatgtaccagaggaagatttatttgaatttgctcttgactacaaaaactttagccgaactgatgcagattacattaagaaatggaaattgtacagttacggcaatagaattaggatatttcggaatcctaagaaaaataatgttttcgattgggaggaagtatgcttgacaagtgcttataaagaactgtttaacaaatatgggattaattaccagcaaggtgatattcgagcactactttgcgagcaatctgacaaggcattttactcgagctttatggccttgatgagtttaatgctacaaatgcggaactcaattactggaagaacagatgtagatttcttgatttcacctgtcaagaattcagatggtatattttatgattcaaggaactatgaagctcaagagaacgctattttgccgaagaatgctgacgccaacggagcatataatatagcacgtaaggtgctttgggctattggacaatttaaaaaggcagaggatgaaaaacttgacaaagtgaagattgcaatttcaaataaggagtggcttgaatatgctcagacaagcgtgaagcataagcggccagcggccacaaagaaggctgggcaagctaagaagaagaaaggttcatatccgtatgatgttcctgattatgcaggatatccatatgatgttcccgactatgctggttcttatccttatgatgtgcctgattacgccggttctccaaagaagaagagaaaggtctga

SEQ ID NO: 68 - DNA, 21 bp, synthetic construct
  misc_feature 1..21: note = 68
  source 1..21: mol_type = other DNA
taatttctactaagtgtagat